European Patent Application EP 4 349 858 A1, published April 10, 2024. Title: CHIMERIC ANTIGEN RECEPTOR SPECIFICALLY BINDING TO CD300C ANTIGEN OR RECEPTOR THEREOF. Applicant: CentricsBio, Inc. The sequence listing filed with the application follows.

SEQUENCE LISTING (442 sequences)

SEQ ID NO: 1 - DNA, 30 bp, Artificial Sequence
  CK1 Heavy Chain CDR1
ttcagccgctatgccatgacctgggttcgc

SEQ ID NO: 2 - DNA, 45 bp, Artificial Sequence
  CK1 Heavy Chain CDR2
agcagcatgagcggcaccggcggcaccacctattatgccgatagc

SEQ ID NO: 3 - DNA, 36 bp, Artificial Sequence
  CK1 Heavy Chain CDR3
tactgtgcccgcggcgcctatggctttgatcattgg

SEQ ID NO: 4 - DNA, 41 bp, Artificial Sequence
  CK1 Light Chain CDR1
tgccgcgccagccagagcatcggcaactatctgaactggta

SEQ ID NO: 5 - DNA, 36 bp, Artificial Sequence
  CK1 Light Chain CDR2
ctgatctatgatgccagcaacctggaaaccggcatc

SEQ ID NO: 6 - DNA, 45 bp, Artificial Sequence
  CK1 Light Chain CDR3
tattattgtcagcagagtagcgccatcccttataccttcggtcag

SEQ ID NO: 7 - protein, 12 aa, Artificial Sequence
  CK1 Heavy Chain CDR1
FTFSRYAMTWVR

SEQ ID NO: 8 - protein, 13 aa, Artificial Sequence
  CK1 Heavy Chain CDR2
SMSGTGGTTYYAD

SEQ ID NO: 9 - protein, 12 aa, Artificial Sequence
  CK1 Heavy Chain CDR3
YCARGAYGFDHW

SEQ ID NO: 10 - protein, 13 aa, Artificial Sequence
  CK1 Light Chain CDR1
CRASQSIGNYLNW

SEQ ID NO: 11 - protein, 10 aa, Artificial Sequence
  CK1 Light Chain CDR2
DASNLETGIP

SEQ ID NO: 12 - protein, 12 aa, Artificial Sequence
  CK1 Light Chain CDR3
YCQQSSAIPYTF

SEQ ID NO: 13 - DNA, 30 bp, Artificial Sequence
  CK2 Heavy Chain CDR1
ttcagcagctatggcatgcattgggttcgc

SEQ ID NO: 14 - DNA, 45 bp, Artificial Sequence
  CK2 Heavy Chain CDR2
agcgccatcagcggcagcggcaccagcatctattatgccgatagc

SEQ ID NO: 15 - DNA, 36 bp, Artificial Sequence
  CK2 Heavy Chain CDR3
tactgtgcccgcggcggcaccgcctttgattattgg

SEQ ID NO: 16 - DNA, 39 bp, Artificial Sequence
  CK2 Light Chain CDR1
tgccgcgccagccagagatcagacaactatctggcctgg

SEQ ID NO: 17 - DNA, 36 bp, Artificial Sequence
  CK2 Light Chain CDR2
ctgatctatgatgccagcaaccgcgccaccggcatc

SEQ ID NO: 18 - DNA, 45 bp, Artificial Sequence
  CK2 Light Chain CDR3
tattattgtcagcagagctatagcaccccttttaccttcggtcag

SEQ ID NO: 19 - protein, 12 aa, Artificial Sequence
  CK2 Heavy Chain CDR1
FTFSSYGMHWVR

SEQ ID NO: 20 - protein, 13 aa, Artificial Sequence
  CK2 Heavy Chain CDR2
AISGSGTSIYYAD

SEQ ID NO: 21 - protein, 12 aa, Artificial Sequence
  CK2 Heavy Chain CDR3
YCARGGTAFDYW

SEQ ID NO: 22 - protein, 13 aa, Artificial Sequence
  CK2 Light Chain CDR1
CRASQRSDNYLAW

SEQ ID NO: 23 - protein, 10 aa, Artificial Sequence
  CK2 Light Chain CDR2
DASNRATGIP

SEQ ID NO: 24 - protein, 12 aa, Artificial Sequence
  CK2 Light Chain CDR3
YCQQSYSTPFTF

SEQ ID NO: 25 - DNA, 30 bp, Artificial Sequence
  CK3 Heavy Chain CDR1
ttcagcagctatgccatcagctgggttcgc

SEQ ID NO: 26 - DNA, 45 bp, Artificial Sequence
  CK3 Heavy Chain CDR2
agcgccaccagcggcagcggccgcgccacctattatgccgatagc

SEQ ID NO: 27 - DNA, 45 bp, Artificial Sequence
  CK3 Heavy Chain CDR3
tactgtgcgcgcgatacctggtgggaaggctattttgatctgtgg

SEQ ID NO: 28 - DNA, 36 bp, Artificial Sequence
  CK3 Light Chain CDR1
tgccaggccagccatatcagcacccatctgaactgg

SEQ ID NO: 29 - DNA, 36 bp, Artificial Sequence
  CK3 Light Chain CDR2
ctgatctatggcgccagcagccgcgccaccggcatc

SEQ ID NO: 30 - DNA, 45 bp, Artificial Sequence
  CK3 Light Chain CDR3
tattattgtcagcagtataacacctatcctcctaccttcggtcag

SEQ ID NO: 31 - protein, 12 aa, Artificial Sequence
  CK3 Heavy Chain CDR1
FTFSSYAISWVR

SEQ ID NO: 32 - protein, 13 aa, Artificial Sequence
  CK3 Heavy Chain CDR2
ATSGSGRATYYAD

SEQ ID NO: 33 - protein, 15 aa, Artificial Sequence
  CK3 Heavy Chain CDR3
YCARDTWWEGYFDLW

SEQ ID NO: 34 - protein, 12 aa, Artificial Sequence
  CK3 Light Chain CDR1
CQASHISTHLNW

SEQ ID NO: 35 - protein, 10 aa, Artificial Sequence
  CK3 Light Chain CDR2
GASSRATGIP

SEQ ID NO: 36 - protein, 12 aa, Artificial Sequence
  CK3 Light Chain CDR3
YCQQYNTYPPTF

SEQ ID NO: 37 - DNA, 33 bp, Artificial Sequence
  CL4 Heavy Chain CDR1
accttcggcagcaactatatgagctgggttcgc

SEQ ID NO: 38 - DNA, 33 bp, Artificial Sequence
  CL4 Heavy Chain CDR2
atcagcggcagcggcaccagcacctattatgcc

SEQ ID NO: 39 - DNA, 27 bp, Artificial Sequence
  CL4 Heavy Chain CDR3
cgcggcatgtggggcatggatgtgtgg

SEQ ID NO: 40 - DNA, 27 bp, Artificial Sequence
  CL4 Light Chain CDR1
ggcaaacatcggcacaccgtgaactgg

SEQ ID NO: 41 - DNA, 30 bp, Artificial Sequence
  CL4 Light Chain CDR2
ctggatagcgaacgccctagcggcgtacct

SEQ ID NO: 42 - DNA, 27 bp, Artificial Sequence
  CL4 Light Chain CDR3
tatgatagcagcagcgtggtgtttggt

SEQ ID NO: 43 - protein, 12 aa, Artificial Sequence
  CL4 Heavy Chain CDR1
FTFGSNYMSWVR

SEQ ID NO: 44 - protein, 13 aa, Artificial Sequence
  CL4 Heavy Chain CDR2
TISGSGTSTYYAD

SEQ ID NO: 45 - protein, 12 aa, Artificial Sequence
  CL4 Heavy Chain CDR3
YCARGMWGMDVW

SEQ ID NO: 46 - protein, 11 aa, Artificial Sequence
  CL4 Light Chain CDR1
CTGKHRHTVNW

SEQ ID NO: 47 - protein, 10 aa, Artificial Sequence
  CL4 Light Chain CDR2
LDSERPSGVP

SEQ ID NO: 48 - protein, 12 aa, Artificial Sequence
  CL4 Light Chain CDR3
YCQSYDSSSVVF

SEQ ID NO: 49 - DNA, 33 bp, Artificial Sequence
  CL5 Heavy Chain CDR1
accttcagcagctatgccatgcattgggttcgc

SEQ ID NO: 50 - DNA, 33 bp, Artificial Sequence
  CL5 Heavy Chain CDR2
atcagcggcggcggctatggcacctattatgcc

SEQ ID NO: 51 - DNA, 30 bp, Artificial Sequence
  CL5 Heavy Chain CDR3
cgcagcaccgtgtgggcctttgatatctgg

SEQ ID NO: 52 - DNA, 30 bp, Artificial Sequence
  CL5 Light Chain CDR1
ggcaacaacatcggcagcaaaagcgtgcat

SEQ ID NO: 53 - DNA, 30 bp, Artificial Sequence
  CL5 Light Chain CDR2
gatgtgagcaaacgccctagcgagcgtcct

SEQ ID NO: 54 - DNA, 30 bp, Artificial Sequence
  CL5 Light Chain CDR3
tttgatagcagcggcacctggatctttggt

SEQ ID NO: 55 - protein, 12 aa, Artificial Sequence
  CL5 Heavy Chain CDR1
FTFSSYAMHWVR

SEQ ID NO: 56 - protein, 13 aa, Artificial Sequence
  CL5 Heavy Chain CDR2
SISGGGYGTYYAD

SEQ ID NO: 57 - protein, 13 aa, Artificial Sequence
  CL5 Heavy Chain CDR3
YCARSTVWAFDIW

SEQ ID NO: 58 - protein, 13 aa, Artificial Sequence
  CL5 Light Chain CDR1
CSGNNIGSKSVHW

SEQ ID NO: 59 - protein, 11 aa, Artificial Sequence
  CL5 Light Chain CDR2
DVSKRPSERPD

SEQ ID NO: 60 - protein, 13 aa, Artificial Sequence
  CL5 Light Chain CDR3
YCQSFDSSGTWIF

SEQ ID NO: 61 - DNA, 27 bp, Artificial Sequence
  CL6 Heavy Chain CDR1
agcagctacggtatgcattgggtcaga

SEQ ID NO: 62 - DNA, 39 bp, Artificial Sequence
  CL6 Heavy Chain CDR2
gcaattagcggtagcggtggtagcacttactacgcagac

SEQ ID NO: 63 - DNA, 45 bp, Artificial Sequence
  CL6 Heavy Chain CDR3
tgcgcagtcagtggtgcaggtcgtggtttcttcgactactgggga

SEQ ID NO: 64 - DNA, 39 bp, Artificial Sequence
  CL6 Light Chain CDR1
tgcagcggtagcagcagcaacattggtagcaactacgtg

SEQ ID NO: 65 - DNA, 24 bp, Artificial Sequence
  CL6 Light Chain CDR2
gacaacaagcgtcctagtggtgtg

SEQ ID NO: 66 - DNA, 33 bp, Artificial Sequence
  CL6 Light Chain CDR3
tgcagcagctacactagcagcagcactgtgatc

SEQ ID NO: 67 - protein, 12 aa, Artificial Sequence
  CL6 Heavy Chain CDR1
FTFSSYGMHWVR

SEQ ID NO: 68 - protein, 13 aa, Artificial Sequence
  CL6 Heavy Chain CDR2
AISGSGGSTYYAD

SEQ ID NO: 69 - protein, 15 aa, Artificial Sequence
  CL6 Heavy Chain CDR3
YCAVSGAGRGFFDYW

SEQ ID NO: 70 - protein, 15 aa, Artificial Sequence
  CL6 Light Chain CDR1
CSGSSSNIGSNYVYW

SEQ ID NO: 71 - protein, 10 aa, Artificial Sequence
  CL6 Light Chain CDR2
EDNKRPSGVP

SEQ ID NO: 72 - protein, 13 aa, Artificial Sequence
  CL6 Light Chain CDR3
YCSSYTSSSTVIF

SEQ ID NO: 73 - DNA, 27 bp, Artificial Sequence
  CL7 Heavy Chain CDR1
agccgctacgcaatgagctgggtcaga

SEQ ID NO: 74 - DNA, 39 bp, Artificial Sequence; identical to SEQ ID NO: 62
  CL7 Heavy Chain CDR2

SEQ ID NO: 75 - DNA, 39 bp, Artificial Sequence
  CL7 Heavy Chain CDR3
tgcgcacgtagcagccagggtatcttcgacatctgggga

SEQ ID NO: 76 - DNA, 33 bp, Artificial Sequence
  CL7 Light Chain CDR1
tgcagtggtaacaatatcggtactagacgcgtg

SEQ ID NO: 77 - DNA, 24 bp, Artificial Sequence
  CL7 Light Chain CDR2
aagaacaaccgtcctagtggtgtg

SEQ ID NO: 78 - DNA, 39 bp, Artificial Sequence
  CL7 Light Chain CDR3
tgcgcagcatgggacgacagcctgagcggtcctgtgttc

SEQ ID NO: 79 - protein, 12 aa, Artificial Sequence
  CL7 Heavy Chain CDR1
FTFSRYAMSWVR

SEQ ID NO: 80 - protein, 13 aa, Artificial Sequence
  CL7 Heavy Chain CDR2
AISGSGGSTYYAD

SEQ ID NO: 81 - protein, 13 aa, Artificial Sequence
  CL7 Heavy Chain CDR3
YCARSSQGIFDIW

SEQ ID NO: 82 - protein, 13 aa, Artificial Sequence
  CL7 Light Chain CDR1
CSGNNIGTRRVHW

SEQ ID NO: 83 - protein, 10 aa, Artificial Sequence
  CL7 Light Chain CDR2
SKNNRPSGVP

SEQ ID NO: 84 - protein, 14 aa, Artificial Sequence
  CL7 Light Chain CDR3
YCAAWDDSLSGPVF

SEQ ID NO: 85 - DNA, 27 bp, Artificial Sequence
  CL8 Heavy Chain CDR1
agcagctacgcaatgagctgggtcaga

SEQ ID NO: 86 - DNA, 39 bp, Artificial Sequence; identical to SEQ ID NO: 62
  CL8 Heavy Chain CDR2

SEQ ID NO: 87 - DNA, 42 bp, Artificial Sequence
  CL8 Heavy Chain CDR3
tgcgcacgtagcggtcgttacgcagacttgacatctggggga

SEQ ID NO: 88 - DNA, 39 bp, Artificial Sequence
  CL8 Light Chain CDR1
tgcagcggtagcaacagcaacatcggtaacaactacgtg

SEQ ID NO: 89 - DNA, 24 bp, Artificial Sequence
  CL8 Light Chain CDR2
aacaacaagcgtcctagtggtgtg

SEQ ID NO: 90 - DNA, 36 bp, Artificial Sequence
  CL8 Light Chain CDR3
tgcagcagctacactagcagcagcactgtgatgttc

SEQ ID NO: 91 - protein, 12 aa, Artificial Sequence
  CL8 Heavy Chain CDR1
FTFSSYAMSWVR

SEQ ID NO: 92 - protein, 13 aa, Artificial Sequence
  CL8 Heavy Chain CDR2
AISGSGGSTYYAD

SEQ ID NO: 93 - protein, 14 aa, Artificial Sequence
  CL8 Heavy Chain CDR3
YCARSGRYADLTSG

SEQ ID NO: 94 - protein, 15 aa, Artificial Sequence
  CL8 Light Chain CDR1
CSGSNSNIGNNYVSW

SEQ ID NO: 95 - protein, 10 aa, Artificial Sequence
  CL8 Light Chain CDR2
DNNKRPSGVP

SEQ ID NO: 96 - protein, 13 aa, Artificial Sequence
  CL8 Light Chain CDR3
YCSSYTSSSTVMF

SEQ ID NO: 97 - DNA, 27 bp, Artificial Sequence
  CL9 Heavy Chain CDR1
agcagctactactggagctgggtcaga

SEQ ID NO: 98 - DNA, 39 bp, Artificial Sequence; identical to SEQ ID NO: 62
  CL9 Heavy Chain CDR2

SEQ ID NO: 99 - DNA, 39 bp, Artificial Sequence
  CL9 Heavy Chain CDR3
tgcgcacgtatcgacgtgtacggtttcgacatctgggga

SEQ ID NO: 100 - DNA, 39 bp, Artificial Sequence
  CL9 Light Chain CDR1
tgcagcggtagcactagcaacatcggtactaactacgtg

SEQ ID NO: 101 - DNA, 24 bp, Artificial Sequence
  CL9 Light Chain CDR2
aacaacaaccgtcctagtggtgtg

SEQ ID NO: 102 - DNA, 33 bp, Artificial Sequence
  CL9 Light Chain CDR3
tgccagacttgggacagcagcactgacgtagtg

SEQ ID NO: 103 - protein, 12 aa, Artificial Sequence
  CL9 Heavy Chain CDR1
FTFSSYYWSWVR

SEQ ID NO: 104 - protein, 13 aa, Artificial Sequence
  CL9 Heavy Chain CDR2
AISGSGGSTYYAD

SEQ ID NO: 105 - protein, 13 aa, Artificial Sequence
  CL9 Heavy Chain CDR3
YCARIDVYGFDIW

SEQ ID NO: 106 - protein, 15 aa, Artificial Sequence
  CL9 Light Chain CDR1
CSGSTSNIGTNYVYW

SEQ ID NO: 107 - protein, 10 aa, Artificial Sequence
  CL9 Light Chain CDR2
DNNNRPSGVP

SEQ ID NO: 108 - protein, 13 aa, Artificial Sequence
  CL9 Light Chain CDR3
YCQTWDSSTDVVF

SEQ ID NO: 109 - DNA, 31 bp, Artificial Sequence
  CL10 Heavy Chain CDR1
tcagcagctacggtatgcattgggtcagaca

SEQ ID NO: 110 - DNA, 43 bp, Artificial Sequence
  CL10 Heavy Chain CDR2
ctgcaattagcggtagcggtggtagcacttactacgcagacag

SEQ ID NO: 111 - DNA, 40 bp, Artificial Sequence
  CL10 Heavy Chain CDR3
actgcgcaagcggttacggtctgatggacgtgtggggaca

SEQ ID NO: 112 - DNA, 43 bp, Artificial Sequence
  CL10 Light Chain CDR1
gctgcactcgtagcagcggtatcatcgcaagcaactacgtgca

SEQ ID NO: 113 - DNA, 27 bp, Artificial Sequence
  CL10 Light Chain CDR2
cgcaacaaccagcgccctagtggtgtg

SEQ ID NO: 114 - DNA, 40 bp, Artificial Sequence
  CL10 Light Chain CDR3
actgcagcagctacgcaggtaacaacaacctggtgttcgg

SEQ ID NO: 115 - protein, 12 aa, Artificial Sequence
  CL10 Heavy Chain CDR1
FTFSSYGMHWVR

SEQ ID NO: 116 - protein, 13 aa, Artificial Sequence
  CL10 Heavy Chain CDR2
AISGSGGSTYYAD

SEQ ID NO: 117 - protein, 12 aa, Artificial Sequence
  CL10 Heavy Chain CDR3
YCASGYGLMDVW

SEQ ID NO: 118 - protein, 15 aa, Artificial Sequence
  CL10 Light Chain CDR1
CTRSSGIIASNYVQW

SEQ ID NO: 119 - protein, 10 aa, Artificial Sequence
  CL10 Light Chain CDR2
RNNQRPSGVP

SEQ ID NO: 120 - protein, 13 aa, Artificial Sequence
  CL10 Light Chain CDR3
YCSSYAGNNNLVF

SEQ ID NO: 121 - DNA, 30 bp, Artificial Sequence
  SK11 Heavy Chain CDR1
ttcagcacctatggcatgcattgggttcgc

SEQ ID NO: 122 - DNA, 42 bp, Artificial Sequence
  SK11 Heavy Chain CDR2
agcgccatcagcggcagcggcggcagcacctattatgccgat

SEQ ID NO: 123 - DNA, 36 bp, Artificial Sequence
  SK11 Heavy Chain CDR3
tactgtgcccgcggcctgagcggccttgattattgg

SEQ ID NO: 124 - DNA, 39 bp, Artificial Sequence
  SK11 Light Chain CDR1
tgccgctccagccagggcatcaccaactatctggcctgg

SEQ ID NO: 125 - DNA, 36 bp, Artificial Sequence; identical to SEQ ID NO: 17
  SK11 Light Chain CDR2

SEQ ID NO: 126 - DNA, 45 bp, Artificial Sequence
  SK11 Light Chain CDR3
tattattgtcagcagagctatagcacccctctgaccttcggtcag

SEQ ID NO: 127 - protein, 12 aa, Artificial Sequence
  SK11 Heavy Chain CDR1
FTFSTYGMHWVR

SEQ ID NO: 128 - protein, 13 aa, Artificial Sequence
  SK11 Heavy Chain CDR2
AISGSGGSTYYAD

SEQ ID NO: 129 - protein, 12 aa, Artificial Sequence
  SK11 Heavy Chain CDR3
YCARGLSGLDYW

SEQ ID NO: 130 - protein, 13 aa, Artificial Sequence
  SK11 Light Chain CDR1
CRSSQGITNYLAW

SEQ ID NO: 131 - protein, 10 aa, Artificial Sequence
  SK11 Light Chain CDR2
DASNRATGIP

SEQ ID NO: 132 - protein, 12 aa, Artificial Sequence
  SK11 Light Chain CDR3
YCQQSYSTPLTF

SEQ ID NO: 133 - DNA, 34 bp, Artificial Sequence
  SK12 Heavy Chain CDR1
ccttcagcagctatgccatgcattgggttcgcca

SEQ ID NO: 134 - DNA, 49 bp, Artificial Sequence
  SK12 Heavy Chain CDR2
tgagcgccatcagcggcagcggcggcgatacctatcatgccgatagcgt

SEQ ID NO: 135 - DNA, 40 bp, Artificial Sequence
  SK12 Heavy Chain CDR3
actactgtacccgcggcctgagcggctttgattattgggg

SEQ ID NO: 136 - DNA, 43 bp, Artificial Sequence
  SK12 Light Chain CDR1
catgccgcgccagccagagcatcagcagctatctgaactggta

SEQ ID NO: 137 - DNA, 40 bp, Artificial Sequence
  SK12 Light Chain CDR2
tgctgatctatgatgccagcaaccgcgcccctggcatccc

SEQ ID NO: 138 - DNA, 49 bp, Artificial Sequence
  SK12 Light Chain CDR3
tgtattattgtcagcagagctatagcatccctatcaccttcggtcaggg

SEQ ID NO: 139 - protein, 12 aa, Artificial Sequence
  SK12 Heavy Chain CDR1
FTFSSYAMHWVR

SEQ ID NO: 140 - protein, 13 aa, Artificial Sequence
  SK12 Heavy Chain CDR2
AISGSGGDTYHAD

SEQ ID NO: 141 - protein, 12 aa, Artificial Sequence
  SK12 Heavy Chain CDR3
YCTRGLSGFDYW

SEQ ID NO: 142 - protein, 13 aa, Artificial Sequence
  SK12 Light Chain CDR1
CRASQSISSYLNW

SEQ ID NO: 143 - protein, 10 aa, Artificial Sequence
  SK12 Light Chain CDR2
DASNRAPGIP

SEQ ID NO: 144 - protein, 12 aa, Artificial Sequence
  SK12 Light Chain CDR3
YCQQSYSIPITF

SEQ ID NO: 145 - DNA, 30 bp, Artificial Sequence
  SK13 Heavy Chain CDR1
ttcagcgattatgccatgagctgggttcgc

SEQ ID NO: 146 - DNA, 42 bp, Artificial Sequence
  SK13 Heavy Chain CDR2
agcatcagcagcagcagcagctatatctactataccgatagc

SEQ ID NO: 147 - DNA, 36 bp, Artificial Sequence
  SK13 Heavy Chain CDR3
tactgtgcccgcggcggctatggctttgattattgg

SEQ ID NO: 148 - DNA, 39 bp, Artificial Sequence
  SK13 Light Chain CDR1
tgccgcgccagccagagcatcagcagctatctgaactgg

SEQ ID NO: 149 - DNA, 36 bp, Artificial Sequence
  SK13 Light Chain CDR2
ctgatctatagcgccagcagccgcccacagggcatc

SEQ ID NO: 150 - DNA, 45 bp, Artificial Sequence
  SK13 Light Chain CDR3
tattattgtcagcagtatgatgatctgccttttaccttcggtcag

SEQ ID NO: 151 - protein, 12 aa, Artificial Sequence
  SK13 Heavy Chain CDR1
FTFSDYAMSWVR

SEQ ID NO: 152 - protein, 13 aa, Artificial Sequence
  SK13 Heavy Chain CDR2
SISSSSSYIYYTD

SEQ ID NO: 153 - protein, 12 aa, Artificial Sequence
  SK13 Heavy Chain CDR3
YCARGGYGFDYW

SEQ ID NO: 154 - protein, 13 aa, Artificial Sequence
  SK13 Light Chain CDR1
CRASQSISSYLNW

SEQ ID NO: 155 - protein, 10 aa, Artificial Sequence
  SK13 Light Chain CDR2
SASSRPQGIP

SEQ ID NO: 156 - protein, 12 aa, Artificial Sequence
  SK13 Light Chain CDR3
YCQQYDDLPFTF

SEQ ID NO: 157 - DNA, 34 bp, Artificial Sequence
  SK14 Heavy Chain CDR1
ccttcagcaactttgcgatcgcctgggttcgcca

SEQ ID NO: 158 - DNA, 46 bp, Artificial Sequence
  SK14 Heavy Chain CDR2
gcgccatcagcggccgcggcaccagcacctattatgccgatagcgt

SEQ ID NO: 159 - DNA, 40 bp, Artificial Sequence
  SK14 Heavy Chain CDR3
actactgtgcccgcggcgtgagcggctttgatagctgggg

SEQ ID NO: 160 - DNA, 43 bp, Artificial Sequence
  SK14 Light Chain CDR1
catgccgcgccagccagagcatcagcagccatctggcctggta

SEQ ID NO: 161 - DNA, 40 bp, Artificial Sequence
  SK14 Light Chain CDR2
tgctgatctatgataccagcaaccgcgccaccggcatccc

SEQ ID NO: 162 - DNA, 49 bp, Artificial Sequence
  SK14 Light Chain CDR3
tgtactattgtcagcagagctatagcaccccttttaccttcggtcaggg

SEQ ID NO: 163 - protein, 12 aa, Artificial Sequence
  SK14 Heavy Chain CDR1
FTFSNFAIAWVR

SEQ ID NO: 164 - protein, 13 aa, Artificial Sequence
  SK14 Heavy Chain CDR2
AISGRGTSTYYAD

SEQ ID NO: 165 - protein, 12 aa, Artificial Sequence
  SK14 Heavy Chain CDR3
YCARGVSGFDSW

SEQ ID NO: 166 - protein, 13 aa, Artificial Sequence
  SK14 Light Chain CDR1
CRASQSISSHLAW

SEQ ID NO: 167 - protein, 10 aa, Artificial Sequence
  SK14 Light Chain CDR2
DTSNRATGIP

SEQ ID NO: 168 - protein, 12 aa, Artificial Sequence
  SK14 Light Chain CDR3
YCQQSYSTPFTF

SEQ ID NO: 169 - DNA, 34 bp, Artificial Sequence; identical to SEQ ID NO: 133
  SK15 Heavy Chain CDR1

SEQ ID NO: 170 - DNA, 49 bp, Artificial Sequence
  SK15 Heavy Chain CDR2
tgagcgccatcaacggcagcggcggcagcacctattatgccgatagcgt

SEQ ID NO: 171 - DNA, 43 bp, Artificial Sequence
  SK15 Heavy Chain CDR3
actactgtgcccgcggcctgcagggctttgattattggggaca

SEQ ID NO: 172 - DNA, 43 bp, Artificial Sequence
  SK15 Light Chain CDR1
catgccaggccagccaggatatcaccaactatctgaactggta

SEQ ID NO: 173 - DNA, 40 bp, Artificial Sequence
  SK15 Light Chain CDR2
tgctgatctatgatgccagcagcctggaaaccggcatccc

SEQ ID NO: 174 - DNA, 49 bp, Artificial Sequence
  SK15 Light Chain CDR3
tgtattattgtcagcagagctatagcacccctatcaccttcggtcaggg

SEQ ID NO: 175 - protein, 12 aa, Artificial Sequence
  SK15 Heavy Chain CDR1
FTFSSYAMHWVR

SEQ ID NO: 176 - protein, 13 aa, Artificial Sequence
  SK15 Heavy Chain CDR2
AINGSGGSTYYAD

SEQ ID NO: 177 - protein, 12 aa, Artificial Sequence
  SK15 Heavy Chain CDR3
YCARGLQGFDYW

SEQ ID NO: 178 - protein, 13 aa, Artificial Sequence
  SK15 Light Chain CDR1
CQASQDITNYLNW

SEQ ID NO: 179 - protein, 10 aa, Artificial Sequence
  SK15 Light Chain CDR2
DASSLETGIP

SEQ ID NO: 180 - protein, 12 aa, Artificial Sequence
  SK15 Light Chain CDR3
YCQQSYSTPITF

SEQ ID NO: 181 - DNA, 34 bp, Artificial Sequence
  SK16 Heavy Chain CDR1
ccttcagcagctatgccatgagctgggttcgcca

SEQ ID NO: 182 - DNA, 49 bp, Artificial Sequence
  SK16 Heavy Chain CDR2
tgagcgccatcaacggcagcggcggcagcaccctgtatgccgatagcgt

SEQ ID NO: 183 - DNA, 40 bp, Artificial Sequence; identical to SEQ ID NO: 159
  SK16 Heavy Chain CDR3

SEQ ID NO: 184 - DNA, 43 bp, Artificial Sequence
  SK16 Light Chain CDR1
catgccgcatcagccagagcatcagcagctatctgaactggta

SEQ ID NO: 185 - DNA, 40 bp, Artificial Sequence
  SK16 Light Chain CDR2
tgctgatctatgatgccagcctgcgcgccaccggcatccc

SEQ ID NO: 186 - DNA, 49 bp, Artificial Sequence
  SK16 Light Chain CDR3
tgtattattgtcagcagagctataaaacccctatcaccttcggtcaggg

SEQ ID NO: 187 - protein, 12 aa, Artificial Sequence
  SK16 Heavy Chain CDR1
FTFSSYAMSWVR

SEQ ID NO: 188 - protein, 13 aa, Artificial Sequence
  SK16 Heavy Chain CDR2
AINGSGGSTLYAD

SEQ ID NO: 189 - protein, 12 aa, Artificial Sequence
  SK16 Heavy Chain CDR3
YCARGVSGFDSW

SEQ ID NO: 190 - protein, 13 aa, Artificial Sequence
  SK16 Light Chain CDR1
CRISQSISSYLNW

SEQ ID NO: 191 - protein, 10 aa, Artificial Sequence
  SK16 Light Chain CDR2
DASLRATGIP

SEQ ID NO: 192 - protein, 13 aa, Artificial Sequence
  SK16 Light Chain CDR3
YYCQQSYKTPITF

SEQ ID NO: 193 - DNA, 34 bp, Artificial Sequence
  SK17 Heavy Chain CDR1
ccttcagcagctattattggagctgggttcgcca

SEQ ID NO: 194 - DNA, 49 bp, Artificial Sequence
  SK17 Heavy Chain CDR2
tgagcaccatcaccggcagcggcggcagcaccgattatgccaacagcgt

SEQ ID NO: 195 - DNA, 40 bp, Artificial Sequence
  SK17 Heavy Chain CDR3
actactgtgccaccggcggcggcatctttgactattgggg

SEQ ID NO: 196 - DNA, 43 bp, Artificial Sequence
  SK17 Light Chain CDR1
catgccaggccagccagaccatcagcaactatctgaactggta

SEQ ID NO: 197 - DNA, 40 bp, Artificial Sequence
  SK17 Light Chain CDR2
tgctgatctatgatgccagcaaccgcgccaccggcatccc

SEQ ID NO: 198 - DNA, 49 bp, Artificial Sequence
  SK17 Light Chain CDR3
tgtattattgtcagcagtacaacagctatcctcctagcttcggtcaggg

SEQ ID NO: 199 - protein, 12 aa, Artificial Sequence
  SK17 Heavy Chain CDR1
FTFSSYYWSWVR

SEQ ID NO: 200 - protein, 13 aa, Artificial Sequence
  SK17 Heavy Chain CDR2
TITGSGGSTDYAN

SEQ ID NO: 201 - protein, 12 aa, Artificial Sequence
  SK17 Heavy Chain CDR3
YCATGGGIFDYW

SEQ ID NO: 202 - protein, 13 aa, Artificial Sequence
  SK17 Light Chain CDR1
CQASQTISNYLNW

SEQ ID NO: 203 - protein, 10 aa, Artificial Sequence
  SK17 Light Chain CDR2
DASNRATGIP

SEQ ID NO: 204 - protein, 12 aa, Artificial Sequence
  SK17 Light Chain CDR3
YCQQYNSYPPSF

SEQ ID NO: 205 - DNA, 34 bp, Artificial Sequence
  SL18 Heavy Chain CDR1
tcaccttcagcgattatcatatgcattgggttcg

SEQ ID NO: 206 - DNA, 34 bp, Artificial Sequence
  SL18 Heavy Chain CDR2
tcagcagcagcggcggctatacctattatgccga

SEQ ID NO: 207 - DNA, 34 bp, Artificial Sequence
  SL18 Heavy Chain CDR3
cccgatcgatacgcctgcctctggattattgggg

SEQ ID NO: 208 - DNA, 37 bp, Artificial Sequence
  SL18 Light Chain CDR1
gcggcaacaacatcggcagcaaaggcgtgcattggta

SEQ ID NO: 209 - DNA, 34 bp, Artificial Sequence
  SL18 Light Chain CDR2
atgaagatagcaaacgccctagcggcgtgcgtga

SEQ ID NO: 210 - DNA, 34 bp, Artificial Sequence
  SL18 Light Chain CDR3
gctatgatagcaccaaaggcgtggtgtttggtgg

SEQ ID NO: 211 - protein, 12 aa, Artificial Sequence
  SL18 Heavy Chain CDR1
FTFSDYHMHWVR

SEQ ID NO: 212 - protein, 13 aa, Artificial Sequence
  SL18 Heavy Chain CDR2
TISSSGGYTYYAE

SEQ ID NO: 213 - protein, 13 aa, Artificial Sequence
  SL18 Heavy Chain CDR3
YCARSIRLPLDYW

SEQ ID NO: 214 - protein, 13 aa, Artificial Sequence
  SL18 Light Chain CDR1
CSGNNIGSKGVHW

SEQ ID NO: 215 - protein, 10 aa, Artificial Sequence
  SL18 Light Chain CDR2
EDSKRPSGVR

SEQ ID NO: 216 - protein, 13 aa, Artificial Sequence
  SL18 Light Chain CDR3
YCQSYDSTKGVVF

SEQ ID NO: 217 - DNA, 34 bp, Artificial Sequence
  CB301_H3L1_A10 Heavy Chain CDR1
tcagcagctacggtatgcattgggtcagacaggc

SEQ ID NO: 218 - DNA, 43 bp, Artificial Sequence; identical to SEQ ID NO: 110
  CB301_H3L1_A10 Heavy Chain CDR2

SEQ ID NO: 219 - DNA, 40 bp, Artificial Sequence
  CB301_H3L1_A10 Heavy Chain CDR3
actgcgtgcgtggttacggtgcaatggacgtgtggggaca

SEQ ID NO: 220 - DNA, 43 bp, Artificial Sequence
  CB301_H3L1_A10 Light Chain CDR1
gctgcactcgtagcagcggtagcatcgcaagcaactacgtgca

SEQ ID NO: 221 - DNA, 31 bp, Artificial Sequence
  CB301_H3L1_A10 Light Chain CDR2
accgcaacaaccagcgccctagtggtgtgcc

SEQ ID NO: 222 - DNA, 40 bp, Artificial Sequence
  CB301_H3L1_A10 Light Chain CDR3
actgcagcagctacactactagcagcactctggtgttcgg

SEQ ID NO: 223 - protein, 12 aa, Artificial Sequence
  CB301_H3L1_A10 Heavy Chain CDR1
FTFSSYGMHWVR

SEQ ID NO: 224 - protein, 13 aa, Artificial Sequence
  CB301_H3L1_A10 Heavy Chain CDR2
AISGSGGSTYYAD

SEQ ID NO: 225 - protein, 12 aa, Artificial Sequence
  CB301_H3L1_A10 Heavy Chain CDR3
YCVRGYGAMDVW

SEQ ID NO: 226 - protein, 15 aa, Artificial Sequence
  CB301_H3L1_A10 Light Chain CDR1
CTRSSGSIASNYVQW

SEQ ID NO: 227 - protein, 10 aa, Artificial Sequence
  CB301_H3L1_A10 Light Chain CDR2
RNNQRPSGVP

SEQ ID NO: 228 - protein, 13 aa, Artificial Sequence
  CB301_H3L1_A10 Light Chain CDR3
YCSSYTTSSTLVF

SEQ ID NO: 229 - DNA, 34 bp, Artificial Sequence
  CB301_H3L1_A12 Heavy Chain CDR1
tcagcagctacgcaatgcattgggtcagacaggc

SEQ ID NO: 230 - DNA, 43 bp, Artificial Sequence; identical to SEQ ID NO: 110
  CB301_H3L1_A12 Heavy Chain CDR2

SEQ ID NO: 231 - DNA, 40 bp, Artificial Sequence
  CB301_H3L1_A12 Heavy Chain CDR3
actgcgcaagcggctacggtctgatggacgtatggggaca

SEQ ID NO: 232 - DNA, 46 bp, Artificial Sequence
  CB301_H3L1_A12 Light Chain CDR1
gctgcactggtactagcagcgacgtgggtaactacaacctggtgag

SEQ ID NO: 233 - DNA, 31 bp, Artificial Sequence
  CB301_H3L1_A12 Light Chain CDR2
acagcaacaaccagcgccctagtggtgtgcc

SEQ ID NO: 234 - DNA, 40 bp, Artificial Sequence
  CB301_H3L1_A12 Light Chain CDR3
actgcagcagctacactggtagcaacgctctgttgttcgg

SEQ ID NO: 235 - protein, 12 aa, Artificial Sequence
  CB301_H3L1_A12 Heavy Chain CDR1
FTFSSYAMHWVR

SEQ ID NO: 236 - protein, 13 aa, Artificial Sequence
  CB301_H3L1_A12 Heavy Chain CDR2
AISGSGGSTYYAD

SEQ ID NO: 237 - protein, 12 aa, Artificial Sequence
  CB301_H3L1_A12 Heavy Chain CDR3
YCASGYGLMDVW

SEQ ID NO: 238 - protein, 16 aa, Artificial Sequence
  CB301_H3L1_A12 Light Chain CDR1
CTGTSSDVGNYNLVSW

SEQ ID NO: 239 - protein, 10 aa, Artificial Sequence
  CB301_H3L1_A12 Light Chain CDR2
SNNQRPSGVP

SEQ ID NO: 240 - protein, 13 aa, Artificial Sequence
  CB301_H3L1_A12 Light Chain CDR3
YCSSYTGSNALLF

SEQ ID NO: 241 - DNA, 31 bp, Artificial Sequence
  CB301_H3L1_E6 Heavy Chain CDR1
tcagcagctacgcaatgagctgggtcagaca

SEQ ID NO: 242 - DNA, 43 bp, Artificial Sequence; identical to SEQ ID NO: 110
  CB301_H3L1_E6 Heavy Chain CDR2

SEQ ID NO: 243 - DNA, 40 bp, Artificial Sequence
  CB301_H3L1_E6 Heavy Chain CDR3
actgcgcacgctggcattacagcttcgactactggggaca

SEQ ID NO: 244 - DNA, 37 bp, Artificial Sequence
  CB301_H3L1_E6 Light Chain CDR1
gctgccgtggtaacaacatcggtagcaagcgtgtgca

SEQ ID NO: 245 - DNA, 31 bp, Artificial Sequence
  CB301_H3L1_E6 Light Chain CDR2
acagctacaaccaccgtcctagcggtgtgcc

SEQ ID NO: 246 - DNA, 43 bp, Artificial Sequence
  CB301_H3L1_E6 Light Chain CDR3
actgcaacacttgggacgacagcctggagggtcctgtgttcgg

SEQ ID NO: 247 - protein, 12 aa, Artificial Sequence
  CB301_H3L1_E6 Heavy Chain CDR1
FTFSSYAMSWVR

SEQ ID NO: 248 - protein, 13 aa, Artificial Sequence
  CB301_H3L1_E6 Heavy Chain CDR2
AISGSGGSTYYAD

SEQ ID NO: 249 - protein, 12 aa, Artificial Sequence
  CB301_H3L1_E6 Heavy Chain CDR3
YCARWHYSFDYW

SEQ ID NO: 250 - protein, 13 aa, Artificial Sequence
  CB301_H3L1_E6 Light Chain CDR1
CRGNNIGSKRVHW

SEQ ID NO: 251 - protein, 10 aa, Artificial Sequence
  CB301_H3L1_E6 Light Chain CDR2
SYNHRPSGVP

SEQ ID NO: 252 - protein, 14 aa, Artificial Sequence
  CB301_H3L1_E6 Light Chain CDR3
YCNTWDDSLEGPVF

SEQ ID NO: 253 - DNA, 31 bp, Artificial Sequence
  CB301_H3L1_F4 Heavy Chain CDR1
tcagcggctacgcaatgagctgggtcagaca

SEQ ID NO: 254 - DNA, 43 bp, Artificial Sequence; identical to SEQ ID NO: 110
  CB301_H3L1_F4 Heavy Chain CDR2

SEQ ID NO: 255 - DNA, 43 bp, Artificial Sequence
  CB301_H3L1_F4 Heavy Chain CDR3
actgcgcacgtagtcctagcggtctgttcgactactggggaca

SEQ ID NO: 256 - DNA, 37 bp, Artificial Sequence
  CB301_H3L1_F4 Light Chain CDR1
gctgcggtggtaacaacatcggtagcaagcgtgtgca

SEQ ID NO: 257 - DNA, 31 bp, Artificial Sequence
  CB301_H3L1_F4 Light Chain CDR2
acaacactagcaacaagcatagcggtgtgcc

SEQ ID NO: 258 - DNA, 37 bp, Artificial Sequence
  CB301_H3L1_F4 Light Chain CDR3
actgcagcagctacctacagcagcactctctgttcgg

SEQ ID NO: 259 - protein, 12 aa, Artificial Sequence
  CB301_H3L1_F4 Heavy Chain CDR1
FTFSGYAMSWVR

SEQ ID NO: 260 - protein, 13 aa, Artificial Sequence
  CB301_H3L1_F4 Heavy Chain CDR2
AISGSGGSTYYAD

SEQ ID NO: 261 - protein, 13 aa, Artificial Sequence
  CB301_H3L1_F4 Heavy Chain CDR3
YCARSPSGLFDYW

SEQ ID NO: 262 - protein, 13 aa, Artificial Sequence
  CB301_H3L1_F4 Light Chain CDR1
CGGNNIGSKRVHW

SEQ ID NO: 263 - protein, 10 aa, Artificial Sequence
  CB301_H3L1_F4 Light Chain CDR2
NTSNKHSGVP

SEQ ID NO: 264 - protein, 12 aa, Artificial Sequence
  CB301_H3L1_F4 Light Chain CDR3
YCSSYLQQHSLF

SEQ ID NO: 265 - DNA, 29 bp, Artificial Sequence
  CB301_H3L1_G11 Heavy Chain CDR1
agcagctacgcaatgagctgggtcagaca

SEQ ID NO: 266 - DNA, 43 bp, Artificial Sequence; identical to SEQ ID NO: 110
  CB301_H3L1_G11 Heavy Chain CDR2

SEQ ID NO: 267 - DNA, 49 bp, Artificial Sequence
  CB301_H3L1_G11 Heavy Chain CDR3
actgcacacgtttcgtgggtgcaatcggtgcattcgactactggggaca

SEQ ID NO: 268 - DNA, 37 bp, Artificial Sequence
  CB301_H3L1_G11 Light Chain CDR1
gctgcagtggtaacaacatcggtagccgtagcgtgca

SEQ ID NO: 269 - DNA, 31 bp, Artificial Sequence; identical to SEQ ID NO: 221
  CB301_H3L1_G11 Light Chain CDR2

SEQ ID NO: 270 - DNA, 43 bp, Artificial Sequence
  CB301_H3L1_G11 Light Chain CDR3
actgcgcagcatgggacgacagcctgagcggtcctgtgttcgg

SEQ ID NO: 271 - protein, 12 aa, Artificial Sequence
  CB301_H3L1_G11 Heavy Chain CDR1
FTFSSYAMSWVR

SEQ ID NO: 272 - protein, 13 aa, Artificial Sequence
  CB301_H3L1_G11 Heavy Chain CDR2
AISGSGGSTYYAD

SEQ ID NO: 273 - protein, 15 aa, Artificial Sequence
  CB301_H3L1_G11 Heavy Chain CDR3
YCTRFVGAIGAFDYW

SEQ ID NO: 274 - protein, 13 aa, Artificial Sequence
  CB301_H3L1_G11 Light Chain CDR1
CSGNNIGSRSVHW

SEQ ID NO: 275 - protein, 10 aa, Artificial Sequence
  CB301_H3L1_G11 Light Chain CDR2
RNNQRPSGVP

SEQ ID NO: 276 - protein, 14 aa, Artificial Sequence
  CB301_H3L1_G11 Light Chain CDR3
YCAAWDDSLSGPVF

SEQ ID NO: 277 - DNA, 31 bp, Artificial Sequence
  CB301_OPALTL_B5 Heavy Chain CDR1
tcagccattacgcaatgagctgggtcagaca

SEQ ID NO: 278 - DNA, 43 bp, Artificial Sequence; identical to SEQ ID NO: 110
  CB301_OPALTL_B5 Heavy Chain CDR2

SEQ ID NO: 279 - DNA, 55 bp, Artificial Sequence
  CB301_OPALTL_B5 Heavy Chain CDR3
actgcgcacgtggttgggacagccctactctgacatacttcgacagctggggaca

SEQ ID NO: 280 - DNA, 43 bp, Artificial Sequence
  CB301_OPALTL_B5 Light Chain CDR1
gctgcagcggtactagcagcaacatcggtaacaacgacgtgag

SEQ ID NO: 281 - DNA, 31 bp, Artificial Sequence
  CB301_OPALTL_B5 Light Chain CDR2
accaggacactaagcgtcctagcggtgtgcc

SEQ ID NO: 282 - DNA, 43 bp, Artificial Sequence; identical to SEQ ID NO: 270
  CB301_OPALTL_B5 Light Chain CDR3

SEQ ID NO: 283 - protein, 12 aa, Artificial Sequence
  CB301_OPALTL_B5 Heavy Chain CDR1
FTFSHYAMSWVR

SEQ ID NO: 284 - protein, 13 aa, Artificial Sequence
  CB301_OPALTL_B5 Heavy Chain CDR2
AISGSGGSTYYAD

SEQ ID NO: 285 - protein, 17 aa, Artificial Sequence
  CB301_OPALTL_B5 Heavy Chain CDR3
YCARGWDSPTLTYFDSW

SEQ ID NO: 286 - protein, 15 aa, Artificial Sequence
  CB301_OPALTL_B5 Light Chain CDR1
CSGTSSNIGNNDVSW

SEQ ID NO: 287 - protein, 10 aa, Artificial Sequence
  CB301_OPALTL_B5 Light Chain CDR2
QDTKRPSGVP

SEQ ID NO: 288 - protein, 14 aa, Artificial Sequence
  CB301_OPALTL_B5 Light Chain CDR3
YCAAWDDSLSGPVF

SEQ ID NO: 289 - DNA, 27 bp, Artificial Sequence
  CB301_OPALTL_E6 Heavy Chain CDR1
agcagctacggtatgcattgggtcaga

SEQ ID NO: 290 - DNA, 39 bp, Artificial Sequence
  CB301_OPALTL_E6 Heavy Chain CDR2
gcaatcagcggtagcggtggttacacttactacgcagac

SEQ ID NO: 291 - DNA, 36 bp, Artificial Sequence
  CB301_OPALTL_E6 Heavy Chain CDR3
tgcgcacgctggcattacagcttcgactactgggga

SEQ ID NO: 292 - DNA, 39 bp, Artificial Sequence
  CB301_OPALTL_E6 Light Chain CDR1
tgcagcggtagcagcagcaacatcggtaacaactacgtg

SEQ ID NO: 293 - DNA, 27 bp, Artificial Sequence
  CB301_OPALTL_E6 Light Chain CDR2
cgcaacaaccagcgccctagtggtgtg

SEQ ID NO: 294 - DNA, 33 bp, Artificial Sequence
  CB301_OPALTL_E6 Light Chain CDR3
tgccagagctacgacaacagcaacgtgctgttc

SEQ ID NO: 295 - protein, 12 aa, Artificial Sequence
  CB301_OPALTL_E6 Heavy Chain CDR1
FTFSSYGMHWVR

SEQ ID NO: 296 - protein, 13 aa, Artificial Sequence
  CB301_OPALTL_E6 Heavy Chain CDR2
AISGSGGYTYYAD

SEQ ID NO: 297 - protein, 12 aa, Artificial Sequence
  CB301_OPALTL_E6 Heavy Chain CDR3
YCARWHYSFDYW

SEQ ID NO: 298 - protein, 15 aa, Artificial Sequence
  CB301_OPALTL_E6 Light Chain CDR1
CSGSSSNIGNNYVSW

SEQ ID NO: 299 - protein, 10 aa, Artificial Sequence
  CB301_OPALTL_E6 Light Chain CDR2
RNNQRPSGVP

SEQ ID NO: 300 - protein, 12 aa, Artificial Sequence
  CB301_OPALTL_E6 Light Chain CDR3
YCQSYDNSNVLF

SEQ ID NO: 301 - DNA, 348 bp, Artificial Sequence
  CK1 Heavy chain variable region
gaagtgcagctgctggaaagtggaggtggactggtgcagcctggcggcagcctgcgcctgagctgtgccgccagcggattcaccttcagccgctatgccatgacctgggttcgccaagcacctggcaaaggcctggaatgggtgagcagcatgagcggcaccggcggcaccacctattatgccgatagcgtgaaaggtcgctttaccatcagccgcgataacagcaaaaacaccctgtatctgcagatgaacagcctgcgcgccgaggacaccgcagtctactactgtgcccgcggcgcctatggctttgatcattggggacaaggtactctggtgaccgtgagcagc

SEQ ID NO: 302 - DNA, 321 bp, Artificial Sequence
  CK1 Light Chain Variable Region
gaaatcgtgctgacccagagccctggcaccctgagcctgagccctggcgaacgcgcaacactgtcatgccgcgccagccagagcatcggcaactatctgaactggtatcagcagaaaccaggtcaggctccacgtctgctgatctatgatgccagcaacctggaaaccggcatccctgatcgcttctcaggatctggaagcggtaccgattttaccctgaccatcagccgcctggaacctgaggactttgccgtgtattattgtcagcagagtagcgccatcccttataccttcggtcagggcactaaagtggaaatcaaa

SEQ ID NO: 303 - protein, 116 aa, Artificial Sequence
  CK1 Heavy Chain Variable Region
EVQLLESGGGLVQPGGSLRLSCAASGFTFSRYAMTWVRQAPGKGLEWVSSMSGTGGTTYYADSVKGRFTISRDNSKNTLYLQMNSLRAEDTAVYYCARGAYGFDHWGQGTLVTVSS

SEQ ID NO: 304 - protein, 107 aa, Artificial Sequence
  CK1 Light Chain Variable Region
EIVLTQSPGTLSLSPGERATLSCRASQSIGNYLNWYQQKPGQAPRLLIYDASNLETGIPDRFSGSGSGTDFTLTISRLEPEDFAVYYCQQSSAIPYTFGQGTKVEIK

SEQ ID NO: 305 - DNA, 348 bp, Artificial Sequence
  CK2 Heavy Chain Variable Region
gaagtgcagctgctggaaagtggaggtggactggtgcagcctggcggcagcctgcgcctgagctgtgccgccagcggattcaccttcagcagctatggcatgcattgggttcgccaagcacctggcaaaggcctggaatgggtgagcgccatcagcggcagcggcaccagcatctattatgccgatagcgtgaaaggccgctttaccatcagccgcgataacagcaaaaacaccctgtatctgcagatgaacagcctgcgcgccgaggacaccgcagtctactactgtgcccgcggcggcaccgcctttgattattggggacaaggtactctggtgaccgtgagcagc

SEQ ID NO: 306 - DNA, 321 bp, Artificial Sequence
  CK2 Light Chain Variable Region
gaaatcgtgctgacccagagccctggcaccctgagcctgagccctggcgaacgcgcaacactgtcatgccgcgccagccagagatcagacaactatctggcctggtatcagcagaaaccaggtcaggctccacgtctgctgatctatgatgccagcaaccgcgccaccggcatccctgatcgcttctcaggatctggaagcggtaccgattttaccctgaccatcagccgcctggaacctgaggactttgccgtgtattattgtcagcagagctatagcaccccttttaccttcggtcagggcactaaagtggaaaccaaa

SEQ ID NO: 307 - protein, 116 aa, Artificial Sequence
  CK2 Heavy Chain Variable Region
EVQLLESGGGLVQPGGSLRLSCAASGFTFSSYGMHWVRQAPGKGLEWVSAISGSGTSIYYADSVKGRFTISRDNSKNTLYLQMNSLRAEDTAVYYCARGGTAFDYWGQGTLVTVSS

SEQ ID NO: 308 - protein, 107 aa, Artificial Sequence
  CK2 Light Chain Variable Region
EIVLTQSPGTLSLSPGERATLSCRASQRSDNYLAWYQQKPGQAPRLLIYDASNRATGIPDRFSGSGSGTDFTLTISRLEPEDFAVYYCQQSYSTPFTFGQGTKVETK

SEQ ID NO: 309 - DNA, 357 bp, Artificial Sequence
  CK3 Heavy Chain Variable Region
cgagtgcagctgctggaaagtggaggtggactggtgcagcctggcggcagcctgcgcctgagctgtgccgccagcggattcaccttcagcagctatgccatcagctgggttcgccaagcacctggcaaaggcctggaatgggtgagcgccaccagcggcagcggccgcgccacctattatgccgatagcgtgaaaggccgctttaccatcagccgcgataacagcaaaaacaccctgtatctgcagatgaacagcctgcgcgccgaggacaccgcagtctactactgtgcgcgcgatacctggtgggaaggctattttgatctgtggggacaaggtactctggtgaccgtgagcagc

SEQ ID NO: 310 - DNA, 318 bp, Artificial Sequence
  CK3 Light Chain Variable Region
gaaatcgtgctgacccagagccctggcaccctgagcctgagccctggcgaacgcgcaacactgtcatgccaggccagccatatcagcacccatctgaactggtatcagcagaaaccaggtcaggctccacgtctgctgatctatggcgccagcagccgcgccaccggcatccctgatcgcttctcaggatctggaagcggtaccgattttaccctgaccatcagccgcctggaacctgaggactttgccgtgtattattgtcagcagtataacacctatcctcctaccttcggtcagggcactaaagtggaaatcaaa

SEQ ID NO: 311 - protein, 119 aa, Artificial Sequence
  CK3 Heavy Chain Variable Region
RVQLLESGGGLVQPGGSLRLSCAASGFTFSSYAISWVRQAPGKGLEWVSATSGSGRATYYADSVKGRFTISRDNSKNTLYLQMNSLRAEDTAVYYCARDTWWEGYFDLWGQGTLVTVSS

SEQ ID NO: 312 - protein, 106 aa, Artificial Sequence
  CK3 Light Chain Variable Region
EIVLTQSPGTLSLSPGERATLSCQASHISTHLNWYQQKPGQAPRLLIYGASSRATGIPDRFSGSGSGTDFTLTISRLEPEDFAVYYCQQYNTYPPTFGQGTKVEIK

SEQ ID NO: 313 - DNA, 348 bp, Artificial Sequence
  CL4 Heavy Chain Variable Region
cgagtgcagctgctggaaagtggaggtggactggtgcagcctggcggcagcctgcgcctgagctgtgccgccagcggattcaccttcggcagcaactatatgagctgggttcgccaagcacctggcaaaggcctggaatgggtgagcaccatcagcggcagcggcaccagcacctattatgccgatagcttgaaaggccgctttaccatcagccgcgataacagcaaaaacaccctgtatctgcagatgaacagcctgcgcgccgaggacaccgcagtctactactgtgcccgcggcatgtggggcatggatgtgtggggacaaggtactctggtgaccgtgagcagc

SEQ ID NO: 314 - DNA, 312 bp, Artificial Sequence
  CL4 Light Chain Variable Region
cagagcgtgctgacccagcctcctagcgcctccggtacaccaggacagcgcgtgactattagctgtaccggcaaacatcggcacaccgtgaactggtaccagctactgcctggaactgcacctaagctgctgatctatctggatagcgaacgccctagcggcgtacctgatcgctttagcggtagcaaatcaggcaccagcgccagcctggccatcagcggccttcgctccgaagatgaagccgattattattgtcagagctatgatagcagcagcgtggtgtttggtggcggtaccaagctgaccgtgctg

SEQ ID NO: 315 - protein, 116 aa, Artificial Sequence
  CL4 Heavy Chain Variable Region
RVQLLESGGGLVQPGGSLRLSCAASGFTFGSNYMSWVRQAPGKGLEWVSTISGSGTSTYYADSLKGRFTISRDNSKNTLYLQMNSLRAEDTAVYYCARGMWGMDVWGQGTLVTVSS

SEQ ID NO: 316 - protein, 104 aa, Artificial Sequence
  CL4 Light Chain Variable Region
QSVLTQPPSASGTPGQRVTISCTGKHRHTVNWYQLLPGTAPKLLIYLDSERPSGVPDRFSGSKSGTSASLAISGLRSEDEADYYCQSYDSSSVVFGGGTKLTVL

SEQ ID NO: 317 - DNA, 351 bp, Artificial Sequence
  CL5 Heavy Chain Variable Region
cgagtgcagctgctggaaagtggaggtggactggtgcagcctggcggcagcctgcgcctgagctgtgccgccagcggattcaccttcagcagctatgccatgcattgggttcgccaagcacctggcaaaggcctggaatgggtgagcagcatcagcggcggcggctatggcacctattatgccgatagcgtgaaaggccgctttaccatcagccgcgataacagcaaaaacaccctgtatctgcagatgaacagcctgcgcgccgaggacaccgcagtctactactgtgcccgcagcaccgtgtgggcctttgatatctggggacaaggtactctggtgaccgtgagcagc

SEQ ID NO: 318 - DNA, 321 bp, Artificial Sequence
  CL5 Light Chain Variable Region
cagagcgtgctgacccagcctcctagcgcctccggtacaccaggacagcgcgtgactattagctgtagcggcaacaacatcggcagcaaaagcgtgcattggtaccagcaactgcctggaactgcacctaagctgctgatctatgatgtgagcaaacgccctagcgagcgtcctgatcgctttagcggtagcaaatcaggcaccagcgccagtctggccatcagcgaccttcgctccgaagatgaagccgattattattgtcagagctttgatagcagcggcacctggatctttggtggcggtaccaagctgaccgtgctg

SEQ ID NO: 319 - protein, 117 aa, Artificial Sequence
  CL5 Heavy Chain Variable Region
RVQLLESGGGLVQPGGSLRLSCAASGFTFSSYAMHWVRQAPGKGLEWVSSISGGGYGTYYADSVKGRFTISRDNSKNTLYLQMNSLRAEDTAVYYCARSTVWAFDIWGQGTLVTVSS

SEQ ID NO: 320 - protein, 107 aa, Artificial Sequence
  CL5 Light Chain Variable Region
QSVLTQPPSASGTPGQRVTISCSGNNIGSKSVHWYQQLPGTAPKLLIYDVSKRPSERPDRFSGSKSGTSASLAISDLRSEDEADYYCQSFDSSGTWIFGGGTKLTVL

SEQ ID NO: 321 - DNA, 357 bp, Artificial Sequence
  CL6 Heavy Chain Variable Region
gaggtgcagctgttggagtctggtggaggcttggtacagcctggaggttctcttcgcctctcctgtgcagcctccggattcactttcagcagctacggtatgcattgggtcagacaggcaccaggtaagggactggagtgggtctctgcaattagcggtagcggtggtagcacttactacgcagacagcgtgaagggtcgcttcaccatctcacgcgacaactccaagaacaccctgtacctgcagatgaacagccttcgcgcagaggacactgccgtgtattactgcgcagtcagtggtgcaggtcgtggtttcttcgactactggggacaaggtactctggtcactgtctcctca

SEQ ID NO: 322 - DNA, 327 bp, Artificial Sequence
  CL6 Light Chain Variable Region
cagtctgtgctgactcagccaccttcagcatctggtactccaggtcagcgcgtcaccatcagctgcagcggtagcagcagcaacattggtagcaactacgtgtactggtatcagcaactcccaggcaccgctcctaagctcctgatttacgaggacaacaagcgtcctagtggtgtgcctgatcgcttttctgggtccaagtctggcacctcagcctctctggctatcagtggacttcgctccgaggacgaggctgactattactgcagcagctacactagcagcagcactgtgatcttcggcggtgggaccaaactgaccgtccta

SEQ ID NO: 323 - protein, 119 aa, Artificial Sequence
  CL6 Heavy Chain Variable Region
EVQLLESGGGLVQPGGSLRLSCAASGFTFSSYGMHWVRQAPGKGLEWVSAISGSGGSTYYADSVKGRFTISRDNSKNTLYLQMNSLRAEDTAVYYCAVSGAGRGFFDYWGQGTLVTVSS

SEQ ID NO: 324 - protein, 109 aa, Artificial Sequence
  CL6 Light Chain Variable Region
QSVLTQPPSASGTPGQRVTISCSGSSSNIGSNYVYWYQQLPGTAPKLLIYEDNKRPSGVPDRFSGSKSGTSASLAISGLRSEDEADYYCSSYTSSSTVIFGGGTKLTVL

SEQ ID NO: 325 - DNA, 351 bp, Artificial Sequence
  CL7 Heavy Chain Variable Region
gaggtgcagctgttggagtctggtggaggcttggtacagcctggaggttctcttcgcctctcctgtgcagcctccggattcactttcagccgctacgcaatgagctgggtcagacaggcaccaggtaagggactggagtgggtctctgcaattagcggtagcggtggtagcacttactacgcagacagcgtgaagggtcgcttcaccatctcacgcgacaactccaagaacaccctgtacctgcagatgaacagccttcgcgcagaggacactgccgtgtattactgcgcacgtagcagccagggtatcttcgacatctggggacaaggtactctggtcactgtctcctca

SEQ ID NO: 326 - DNA, 324 bp, Artificial Sequence
  CL7 Light Chain Variable Region
cagtctgtgctgactcagccaccttcagcatctggtactccaggtcagcgcgtcaccatcagctgcagtggtaacaatatcggtactagacgcgtgcattggtatcagcaactcccagacaccgctcctaagctcctgatttacagtaagaacaaccgtcctagtggtgtgcctgatcgcttttctgggtccaagtctggcacctcagcctctctggctatcagtggacttcgctccgaggacgaggctgactattactgcgcagcatgggacgacagcctgagcggtcctgtgttcggcggtgggaccaaactgaccgtccta

SEQ ID NO: 327 - protein, 117 aa, Artificial Sequence
  CL7 Heavy Chain Variable Region
EVQLLESGGGLVQPGGSLRLSCAASGFTFSRYAMSWVRQAPGKGLEWVSAISGSGGSTYYADSVKGRFTISRDNSKNTLYLQMNSLRAEDTAVYYCARSSQGIFDIWGQGTLVTVSS

SEQ ID NO: 328 - protein, 108 aa, Artificial Sequence
  CL7 Light Chain Variable Region
QSVLTQPPSASGTPGQRVTISCSGNNIGTRRVHWYQQLPDTAPKLLIYSKNNRPSGVPDRFSGSKSGTSASLAISGLRSEDEADYYCAAWDDSLSGPVFGGGTKLTVL

SEQ ID NO: 329 - DNA, 354 bp, Artificial Sequence
  CL8 Heavy Chain Variable Region
gaggtgcagctgttggagtctggtggaggcttggtacagcctggaggttctcttcgcctctcctgtgcagcctccggattcactttcagcagctacgcaatgagctgggtcagacaggcaccaggtaagggactggagtgggtctctgcaattagcggtagcggtggtagcacttactacgcagacagcgtgaagggtcgcttcaccatctcacgcaacaactccaagaacaccctgtacctgcagatgaacagccttcgcgcagaggacactgccgtgtattactgcgcacgtagcggtcgttacgcagacttgacatctgggggacaaggtactctggtcactgtctcctca

SEQ ID NO: 330 - DNA, 327 bp, Artificial Sequence
  CL8 Light Chain Variable Region
cagtctgtgctgactcagccaccttcagcatctggtactccaggtcagcgcgtcaccatcagctgcagcggtagcaacagcaacatcggtaacaactacgtgagctggtatcagcaactcccagacacccctcctaagctcctgatttacgacaacaacaagcgtcctagtggtgtgcctgatcgcttttctgggtccaagtctggcacctcagcctctctggctatcagtggacttcgctccgaggacgaggctgactattactgcagcagctacactagcagcagcactgtgatgttcggcggtgggaccaaactgaccgtccta

SEQ ID NO: 331 - protein, 118 aa, Artificial Sequence
  CL8 Heavy Chain Variable Region
EVQLLESGGGLVQPGGSLRLSCAASGFTFSSYAMSWVRQAPGKGLEWVSAISGSGGSTYYADSVKGRFTISRNNSKNTLYLQMNSLRAEDTAVYYCARSGRYADLTSGGQGTLVTVSS

SEQ ID NO: 332 - protein, 109 aa, Artificial Sequence
  CL8 Light Chain Variable Region
QSVLTQPPSASGTPGQRVTISCSGSNSNIGNNYVSWYQQLPDTPPKLLIYDNNKRPSGVPDRFSGSKSGTSASLAISGLRSEDEADYYCSSYTSSSTVMFGGGTKLTVL

SEQ ID NO: 333 - DNA, 351 bp, Artificial Sequence
  CL9 Heavy Chain Variable Region
gaggtgcagctgttggagtctggtggaggcttggtacagcctggaggttctcttcgcctctcctgtgcagcctccggattcactttcagcagctactactggagctgggtcagacaggcaccaggtaagggactggagtgggtctctgcaattagcggtagcggtggtagcacttactacgcagacagcgtgaagggtcgcttcaccatctcacgcgacaactccaagaacaccctgtacctgcagatgaacagccttcgcgcagaggacactgccgtgtattactgcgcacgtatcgacgtgtacggtttcgacatctggggacaaggtactctggtcactgtctcctca

SEQ ID NO: 334 - DNA, 327 bp, Artificial Sequence
  CL9 Light Chain Variable Region
cagtctgtgctgactcagccaccttcagcatctggtactccaggtcagcgcgtcaccatcagctgcagcggtagcactagcaacatcggtactaactacgtgtactggtatcagcaactcccaggcaccgctcctaagctcctgatttacgacaacaacaaccgtcctagtggtgtgcctgatcgcttttctgggtccaagtctggcacctcagcctctctggctatcagtggacttcgctccgaggacgaggctgactattactgccagacttgggacagcagcactgacgtagtgttcggcggtgggaccaaactgaccgtccta

SEQ ID NO: 335 - protein, 117 aa, Artificial Sequence
  CL9 Heavy Chain Variable Region
EVQLLESGGGLVQPGGSLRLSCAASGFTFSSYYWSWVRQAPGKGLEWVSAISGSGGSTYYADSVKGRFTISRDNSKNTLYLQMNSLRAEDTAVYYCARIDVYGFDIWGQGTLVTVSS

SEQ ID NO: 336 - protein, 109 aa, Artificial Sequence
  CL9 Light Chain Variable Region
QSVLTQPPSASGTPGQRVTISCSGSTSNIGTNYVYWYQQLPGTAPKLLIYDNNNRPSGVPDRFSGSKSGTSASLAISGLRSEDEADYYCQTWDSSTDVVFGGGTKLTVL

SEQ ID NO: 337 - DNA, 348 bp, Artificial Sequence
  CL10 Heavy Chain Variable Region
gaggtgcagctgttggagtctggtggaggcttggtacagcctggaggttctcttcgcctctcctgtgcagcctccggattcactttcagcagctacggtatgcattgggtcagacaggcaccaggtaagggactggagtgggtctctgcaattagcggtagcggtggtagcacttactacgcagacagcgtgaagggtcgcttcaccatctcacgcgacaactccaagaacaccctgtacctgcagatgaacagccttcgcgcagaggacactgccgtgtattactgcgcaagcggttacggtctgatggacgtgtggggacaaggtactctggtcactgtctcctca

SEQ ID NO: 338 - DNA, 324 bp, Artificial Sequence
  CL10 Light Chain Variable Region
tctgtgctgactcagccaccttcagcatctggtactccaggtcagcgcgtcaccatcagctgcactcgtagcagcggtatcatcgcaagcaactacgtgcagtggtatcagcaactcccaggcaccgctcctaagctcctgatttaccgcaacaaccagcgccctagtggtgtgcctgatcgcttttctgggtccaagtctggcacctcagcctctctggctatcagtggacttcgctccgaggacgaggctgactattactgcagcagctacgcaggtaacaacaacctggtgttcggcggtgggaccaaactgaccgtccta

SEQ ID NO: 339 - protein, 116 aa, Artificial Sequence
  CL10 Heavy Chain Variable Region
EVQLLESGGGLVQPGGSLRLSCAASGFTFSSYGMHWVRQAPGKGLEWVSAISGSGGSTYYADSVKGRFTISRDNSKNTLYLQMNSLRAEDTAVYYCASGYGLMDVWGQGTLVTVSS

SEQ ID NO: 340 - protein, 109 aa, Artificial Sequence
  CL10 Light Chain Variable Region
QSVLTQPPSASGTPGQRVTISCTRSSGIIASNYVQWYQQLPGTAPKLLIYRNNQRPSGVPDRFSGSKSGTSASLAISGLRSEDEADYYCSSYAGNNNLVFGGGTKLTVL

SEQ ID NO: 341 - DNA, 348 bp, Artificial Sequence
  SK11 Heavy Chain Variable Region
cgagtgcagctgctggaaagtggaggtggactggtgcagcctggcggcagcctgcgcctgagctgtgccgccagcggattcaccttcagcacctatggcatgcattgggttcgccaagcacctggcaaaggcctggaatgggtgagcgccatcagcggcagcggcggcagcacctattatgccgatagcgtgaaaggccgctttaccatcagccgcgataacagcaaaaacaccctgtatctgcagatgaacagcctgcgcgccgaggacaccgcagtctactactgtgcccgcggcctgagcggccttgattattggggacaaggtactctggtgaccgtgagcagc

SEQ ID NO: 342 - DNA, 321 bp, Artificial Sequence
  SK11 Light Chain Variable Region
gaaatcgtgctgacccagagccctggcaccctgagcctgagccctggcgaacgcgcaacactgtcatgccgctccagccagggcatcaccaactatctggcctggtatcagcagaaaccaggtcaggctccacgtctgctgatctatgatgccagcaaccgcgccaccggcatccctgatcgcttctcaggatctggaagcggtaccgattttaccctgaccatcagccgcctggaacctgaggactttgccgtgtattattgtcagcagagctatagcacccctctgaccttcggtcagggcactaaagtggaaatcaaa

SEQ ID NO: 343 - protein, 116 aa, Artificial Sequence
  SK11 Heavy Chain Variable Region
RVQLLESGGGLVQPGGSLRLSCAASGFTFSTYGMHWVRQAPGKGLEWVSAISGSGGSTYYADSVKGRFTISRDNSKNTLYLQMNSLRAEDTAVYYCARGLSGLDYWGQGTLVTVSS

SEQ ID NO: 344 - protein, 107 aa, Artificial Sequence
  SK11 Light Chain Variable Region
EIVLTQSPGTLSLSPGERATLSCRSSQGITNYLAWYQQKPGQAPRLLIYDASNRATGIPDRFSGSGSGTDFTLTISRLEPEDFAVYYCQQSYSTPLTFGQGTKVEIK

SEQ ID NO: 345 - DNA, 348 bp, Artificial Sequence
  SK12 Heavy Chain Variable Region
cgagtgcagctgctggaaagtggaggtggactggtgcagcctggcggcagcctgcgcctgagctgtgccgccagcggattcaccttcagcagctatgccatgcattgggttcgccaagcacctggcaaaggcctggaatgggtgagcgccatcagcggcagcggcggcgatacctatcatgccgatagcgtgaaaggccgctttaccatcagccgcgataacagcaaaaacaccctgtatctgcagatgaacagcctgcgcgccgaggacaccgcagtctactactgtacccgcggcctgagcggctttgattattggggacaaggtactctggtgaccgtgagcagc

SEQ ID NO: 346 - DNA, 321 bp, Artificial Sequence
  SK12 Light Chain Variable Region
gaaatcgtgctgacccagagccctggcaccctgagcctgagccctggcgaacgcgcaacactgtcatgccgcgccagccagagcatcagcagctatctgaactggtatcagcagaaaccaggtcaggctccacgtctgctgatctatgatgccagcaaccgcgcccctggcatccctgatcgcttctcaggatctggaagcggtaccgattttaccctgaccatcagccgcctggaacctgaggactttgccgtgtattattgtcagcagagctatagcatccctatcaccttcggtcagggcactaaagtggaaatcaaa

SEQ ID NO: 347 - protein, 116 aa, Artificial Sequence
  SK12 Heavy Chain Variable Region
RVQLLESGGGLVQPGGSLRLSCAASGFTFSSYAMHWVRQAPGKGLEWVSAISGSGGDTYHADSVKGRFTISRDNSKNTLYLQMNSLRAEDTAVYYCTRGLSGFDYWGQGTLVTVSS

SEQ ID NO: 348 - protein, 110 aa, Artificial Sequence
  SK12 Light Chain Variable Region
EIVLTQSPGTLSLSPGERATLSCRASQSISSYLNWYQQKPGQAPRLLIYDASNRAPGIPDRFSGSGSGTDFTLTISRLEPEDFAVYYCQQSYSIPITFGQGTKVEIKFSD

SEQ ID NO: 349 - DNA, 348 bp, Artificial Sequence
  SK13 Heavy Chain Variable Region
cgagtgcagctgctggaaagtggaggtggactggtgcagcctggcggcagcctgcgcctgagctgtgccgccagcggattcaccttcagcgattatgccatgagctgggttcgccaagcacctggcaaaggcctggaatgggtgagcagcatcagcagcagcagcagctatatctactataccgatagcgtgaaaggccgctttaccatcagccgcgataacagcaaaaacaccctgtatctgcagatgaacagcctgcgcgccgaggacaccgcagtctactactgtgcccgcggcggctatggctttgattattggggacaaggtaccctggtgaccgtgagcagc

SEQ ID NO: 350 - DNA, 321 bp, Artificial Sequence
  SK13 Light Chain Variable Region
gaaatcgtgctgacccagagccctggcaccctgagcctgagccctggcgaacgcgcaacactgtcatgccgcgccagccagagcatcagcagctatctgaactggtatcagcagaaaccaggtcaggctccacgtctgctgatctatagcgccagcagccgcccacagggcatccccgatcgcttctcaggatctggaagcggtaccgattttaccctgaccatcagccgcctggaacctgaggactttgccgtgtattattgtcagcagtatgatgatctgccttttaccttcggtcagggcactaaagtggaaatcaaa

SEQ ID NO: 351 - protein, 116 aa, Artificial Sequence
  SK13 Heavy Chain Variable Region
RVQLLESGGGLVQPGGSLRLSCAASGFTFSDYAMSWVRQAPGKGLEWVSSISSSSSYIYYTDSVKGRFTISRDNSKNTLYLQMNSLRAEDTAVYYCARGGYGFDYWGQGTLVTVSS

SEQ ID NO: 352 - protein, 107 aa, Artificial Sequence
  SK13 Light Chain Variable Region
EIVLTQSPGTLSLSPGERATLSCRASQSISSYLNWYQQKPGQAPRLLIYSASSRPQGIPDRFSGSGSGTDFTLTISRLEPEDFAVYYCQQYDDLPFTFGQGTKVEIK

SEQ ID NO: 353 - DNA, 346 bp, Artificial Sequence
  SK14 Heavy Chain Variable Region
gaagtgcagctgctggaaagtggaggtggactggtgcagcctggcggcagcctgcgcctgagctgtgccgccagcggattcaccttcagcaactttgcgatcgcctgggttcgccaagcacctggcaaaggcctggaatgggtgagcgccatcagcggccgcggcaccagcacctattatgccgatagcgtgaaaggccgctttaccatcagccgcgataacagcaaaaacaccctgtatctgcagatgaacagcctgcgcgccgaggacaccgcagtctactactgtgcccgcggcgtgagcggctttgatagctggggacaaggtactctggtgaccgtgagca

SEQ ID NO: 354 - DNA, 321 bp, Artificial Sequence
  SK14 Light Chain Variable Region
gaaatcgtgctgacccagagccctggcaccctgagcctgagccctggcgaacgcgcaacactgtcatgccgcgccagccagagcatcagcagccatctggcctggtatcagcagaaaccaggtcaggctccacgtctgctgatctatgataccagcaaccgcgccaccggcatccctgatcgcttctcaggatctgggagcggtaccgattttaccctgaccatcagccgcctggaacctgaggactttgccgtgtactattgtcagcagagctatagcaccccttttaccttcggtcagggcactaaagtggaaatcaaa

SEQ ID NO: 355 - protein, 116 aa, Artificial Sequence
  SK14 Heavy Chain Variable Region
EVQLLESGGGLVQPGGSLRLSCAASGFTFSNFAIAWVRQAPGKGLEWVSAISGRGTSTYYADSVKGRFTISRDNSKNTLYLQMNSLRAEDTAVYYCARGVSGFDSWGQGTLVTVSS

SEQ ID NO: 356 - protein, 107 aa, Artificial Sequence
  SK14 Light Chain Variable Region
EIVLTQSPGTLSLSPGERATLSCRASQSISSHLAWYQQKPGQAPRLLIYDTSNRATGIPDRFSGSGSGTDFTLTISRLEPEDFAVYYCQQSYSTPFTFGQGTKVEIK

SEQ ID NO: 357 - DNA, 349 bp, Artificial Sequence
  SK15 Heavy Chain Variable Region
cgagtgcagctgctggaaagtggaggtggactggtgcagcctggcggcagcctgcgcctgagctgtgccgccagcggattcaccttcagcagctatgccatgcattgggttcgccaagcacctggcaaaggcctggaatgggtgagcgccatcaacggcagcggcggcagcacctattatgccgatagcgtgaaaggccgctttaccatcagccgcgataacagcaaaaacaccctgtatctgcagacgaacagcctgcgcgccgaggacaccgcagtctactactgtgcccgcggcctgcagggctttgattattggggacaaggtactctggtgaccgtgagcagca

SEQ ID NO: 358 - DNA, 321 bp, Artificial Sequence
  SK15 Light Chain Variable Region
gaaatcgtgctgacccagagccctggcaccctgagcctgagccctggcgaacgcgcaacactgtcatgccaggccagccaggatatcaccaactatctgaactggtatcagcagaaaccaggtcaggctccacgtctgctgatctatgatgccagcagcctggaaaccggcatccctgatcgtttctcaggatctggaagcggtaccgattttaccctgaccatcagccgcctggaacctgaggactttgccgtgtattattgtcagcagagctatagcacccctatcaccttcggtcagggcactaaagtggaaatcaaa

SEQ ID NO: 359 - protein, 116 aa, Artificial Sequence
  SK15 Heavy Chain Variable Region
RVQLLESGGGLVQPGGSLRLSCAASGFTFSSYAMHWVRQAPGKGLEWVSAINGSGGSTYYADSVKGRFTISRDNSKNTLYLQTNSLRAEDTAVYYCARGLQGFDYWGQGTLVTVSS

SEQ ID NO: 360 - protein, 107 aa, Artificial Sequence
  SK15 Light Chain Variable Region
EIVLTQSPGTLSLSPGERATLSCQASQDITNYLNWYQQKPGQAPRLLIYDASSLETGIPDRFSGSGSGTDFTLTISRLEPEDFAVYYCQQSYSTPITFGQGTKVEIK

SEQ ID NO: 361 - DNA, 349 bp, Artificial Sequence
  SK16 Heavy Chain Variable Region
cgagtgcagctgctggaaagtggaggtggactggtgcagcctggcggcagcctgcgcctgagctgtgccgccagcggattcaccttcagcagctatgccatgagctgggttcgccaagcacctggcaaaggcctggaatgggtgagcgccatcaacggcagcggcggcagcaccctgtatgccgatagcgtgaaaggccgctttaccatcagccgcgataacagcaaaaacaccctgtatctgcagatgaacagcctgcgcgccgaggacaccgcagtctactactgtgcccgcggcgtgagcggctttgatagctggggacaaggtactctggtgaccgtgagcagcg

SEQ ID NO: 362 - DNA, 321 bp, Artificial Sequence
  SK16 Light Chain Variable Region
gaaatcgtgctgacccagagccctggcaccctgagcctgagccctggcgaacgcgcaacactgtcatgccgcatcagccagagcatcagcagctatctgaactggtatcagcagaaaccaggtcaggctccacgtctgctgatctatgatgccagcctgcgcgccaccggcatccctgatcgcttctcaggatctggaagcggtaccgattttaccctgaccatcagccgcctggaacctgaggactttgccgtgtattattgtcagcagagctataaaacccctatcaccttcggtcagggcactaaagtggaaatcaaa

SEQ ID NO: 363 - protein, 116 aa, Artificial Sequence
  SK16 Heavy Chain Variable Region
RVQLLESGGGLVQPGGSLRLSCAASGFTFSSYAMSWVRQAPGKGLEWVSAINGSGGSTLYADSVKGRFTISRDNSKNTLYLQMNSLRAEDTAVYYCARGVSGFDSWGQGTLVTVSS

SEQ ID NO: 364 - protein, 107 aa, Artificial Sequence
  SK16 Light Chain Variable Region
EIVLTQSPGTLSLSPGERATLSCRISQSISSYLNWYQQKPGQAPRLLIYDASLRATGIPDRFSGSGSGTDFTLTISRLEPEDFAVYYCQQSYKTPITFGQGTKVEIK

SEQ ID NO: 365 - DNA, 349 bp, Artificial Sequence
  SK17 Heavy Chain Variable Region
gaagtgcagctgctggaaagtggaggtggactggtgcagcctggcggcagcctgcgcctgagctgtgccgccagcggattcaccttcagcagctattattggagctgggttcgccaagcacctggcaaaggcctggaatgggtgagcaccatcaccggcagcggcggcagcaccgattatgccaacagcgtgaaaggccgctttaccatcagccgcgataacagcaaaaacaccctgtatctgcagatgaacagcctgcgcgccgaggacaccgcagtctactactgtgccaccggcggcggcatctttgactattggggacaaggtactctggtgaccgtgagcagcg

SEQ ID NO: 366 - DNA, 321 bp, Artificial Sequence
  SK17 Light Chain Variable Region
gaaatcgtgctgacccagagccctggcaccctgagcctgagccctggcgaacgcgcaacactgtcatgccaggccagccagaccatcagcaactatctgaactggtatcagcagaaaccaggtcaggctccacgtctgctgatctatgatgccagcaaccgcgccaccggcatccctgatcgcttctcaggatctggaagcggtaccgattttaccctgaccatcagccgcctggaacctgaggactttgccgtgtattattgtcagcagtacaacagctatcctcctagcttcggtcagggcactaaagtggaaatcaaa

SEQ ID NO: 367 - protein, 116 aa, Artificial Sequence
  SK17 Heavy Chain Variable Region
EVQLLESGGGLVQPGGSLRLSCAASGFTFSSYYWSWVRQAPGKGLEWVSTITGSGGSTDYANSVKGRFTISRDNSKNTLYLQMNSLRAEDTAVYYCATGGGIFDYWGQGTLVTVSS

SEQ ID NO: 368 - protein, 107 aa, Artificial Sequence
  SK17 Light Chain Variable Region
EIVLTQSPGTLSLSPGERATLSCQASQTISNYLNWYQQKPGQAPRLLIYDASNRATGIPDRFSGSGSGTDFTLTISRLEPEDFAVYYCQQYNSYPPSFGQGTKVEIK

SEQ ID NO: 369 - DNA, 352 bp, Artificial Sequence
  SL18 Heavy Chain Variable Region
cgagtgcagctgctggaaagtggaggtggactggtgcagcctggcggcagcctgcgcctgagctgtgccgccagcggattcaccttcagcgattatcatatgcattgggttcgccaagcacctggcaaaggcctggaatgggtgagcaccatcagcagcagcggcggctatacctattatgccgaaagcgtgaaaagccgctttaccatcagccgcgataacagcaaaaacaccctgtatctgcagatgaacagcctgcgcgccgaggacaccgcagtctactactgtgcccgatcgatacgcctgcctctggattattggggacaaggtactctggtgaccgtgagcagca

SEQ ID NO: 370 - DNA, 321 bp, Artificial Sequence
  SL18 Light Chain Variable Region
cagagcgtgctgacccagcctcctagcgcctccggtacaccaggacagcgcgtgactattagctgtagcggcaacaacatcggcagcaaaggcgtgcattggtatcagcaactgcctggaactgcacctaagctgctgatctatgaagatagcaaacgccctagcggcgtgcgtgatcgctttagcggtagcaaatcaggcaccagcgccagcctggccatcagcggccttcgctccgaagatgaagccgattattattgtcagagctatgatagcaccaaaggcgtggtgtttggtggcggtaccaagctgaccgtgctg

SEQ ID NO: 371 - protein, 117 aa, Artificial Sequence
  SL18 Heavy Chain Variable Region
RVQLLESGGGLVQPGGSLRLSCAASGFTFSDYHMHWVRQAPGKGLEWVSTISSSGGYTYYAESVKSRFTISRDNSKNTLYLQMNSLRAEDTAVYYCARSIRLPLDYWGQGTLVTVSS

SEQ ID NO: 372 - protein, 107 aa, Artificial Sequence
  SL18 Light Chain Variable Region
QSVLTQPPSASGTPGQRVTISCSGNNIGSKGVHWYQQLPGTAPKLLIYEDSKRPSGVRDRFSGSKSGTSASLAISGLRSEDEADYYCQSYDSTKGVVFGGGTKLTVL

SEQ ID NO: 373 - DNA, 348 bp, Artificial Sequence
  CB301_H3L1_A10 Heavy Chain Variable Region
gaggtgcagctgttggagtctggtggaggcttggtacagtctggaggttctcttcgcctctcctgtgcagcctccggattcactttcagcagctacggtatgcattgggtcagacaggcaccaggtaagggactggagtgggtctctgcaattagcggtagcggtggtagcacttactacgcagacagcgtgaagggtcgcttcaccatctcacgcgacaactccaagaacaccctgtacctgcagatgaacagccttcgcgcagaggacactgccgtgtattactgcgtgcgtggttacggtgcaatggacgtgtggggacaaggtactctggtcactgtctcctca

SEQ ID NO: 374 - DNA, 327 bp, Artificial Sequence
  CB301_H3L1_A10 Light Chain Variable Region
cagtctgtgctgactcagccaccttcagcatctggtactccaggtcagcgcgtcaccatcagctgcactcgtagcagcggtagcatcgcaagcaactacgtgcagtggtatcagcaactcccaggcaccgctcctaagctcctgatttaccgcaacaaccagcgccctagtggtgtgcctgatcgcttttctgggtccaagtctggcacctcagcctctctggctatcagtggacttcgctccgaggacgaggctgactattactgcagcagctacactactagcagcactctggtgttcggcggtgggaccaaactgaccgtccta

SEQ ID NO: 375 - protein, 116 aa, Artificial Sequence
  CB301_H3L1_A10 Heavy Chain Variable Region
EVQLLESGGGLVQSGGSLRLSCAASGFTFSSYGMHWVRQAPGKGLEWVSAISGSGGSTYYADSVKGRFTISRDNSKNTLYLQMNSLRAEDTAVYYCVRGYGAMDVWGQGTLVTVSS

SEQ ID NO: 376 - protein, 109 aa, Artificial Sequence
  CB301_H3L1_A10 Light Chain Variable Region
QSVLTQPPSASGTPGQRVTISCTRSSGSIASNYVQWYQQLPGTAPKLLIYRNNQRPSGVPDRFSGSKSGTSASLAISGLRSEDEADYYCSSYTTSSTLVFGGGTKLTVL

SEQ ID NO: 377 - DNA, 348 bp, Artificial Sequence
  CB301_H3L1_A12 Heavy Chain Variable Region
gaggtgcagctgttggagtctggtggaggcttggtacagcctggaggttctcttcgcctctcctgtgcagcctccggattcactttcagcagctacgcaatgcattgggtcagacaggcaccaggtaagggactggagtgggtctctgcaattagcggtagcggtggtagcacttactacgcagacagcgtgaagggtcgcttcaccatctcacgcgacaactccaagaacaccctgtacctgcagatgaacagccttcgcgcaaaggacactgccgtgtattactgcgcaagcggctacggtctgatggacgtatggggacaaggtactctggtcactgtctcctca

SEQ ID NO: 378 - DNA, 330 bp, Artificial Sequence
  CB301_H3L1_A12 Light Chain Variable Region
cagtctgtgctgactcagccaccttcagcatctggtactccaggtcagcgcgtcaccatcagctgcactggtactagcagcgacgtgggtaactacaacctggtgagctggtatcagcaactcccaggcaccgctcctaagctcctgatttacagcaacaaccagcgccctagtggtgtgcctgatcgcttttctgggtccaagtctggcacctcagcctctctggctatcagtggacttcgctccgaggacgaggctgactattactgcagcagctacactggtagcaacgctctgttgttcggcggtgggaccaaactgaccgtccta

SEQ ID NO: 379 - protein, 116 aa, Artificial Sequence
  CB301_H3L1_A12 Heavy Chain Variable Region
EVQLLESGGGLVQPGGSLRLSCAASGFTFSSYAMHWVRQAPGKGLEWVSAISGSGGSTYYADSVKGRFTISRDNSKNTLYLQMNSLRAKDTAVYYCASGYGLMDVWGQGTLVTVSS

SEQ ID NO: 380 - protein, 110 aa, Artificial Sequence
  CB301_H3L1_A12 Light Chain Variable Region
QSVLTQPPSASGTPGQRVTISCTGTSSDVGNYNLVSWYQQLPGTAPKLLIYSNNQRPSGVPDRFSGSKSGTSASLAISGLRSEDEADYYCSSYTGSNALLFGGGTKLTVL

SEQ ID NO: 381 - DNA, 348 bp, Artificial Sequence
  CB301_H3L1_E6 Heavy Chain Variable Region
gaggtgcagctgttggagtctggtggaggcttggtacagcctggaggttctcttcgcctctcctgtgcagcctccggattcactttcagcagctacgcaatgagctgggtcagacaggcaccaggtaagggactggagtgggtctctgcaattagcggtagcggtggtagcacttactacgcagacagcgtgaagggtcgcttcaccatctcacgcgacaactccaagaacaccctgtacctgcagatgaacagccttcgcgcagaggacactgccgtgtattactgcgcacgctggcattacagcttcgactactggggacaaggtactctggtcactgtctcctca

SEQ ID NO: 382 - DNA, 324 bp, Artificial Sequence
  CB301_H3L1_E6 Light Chain Variable Region
cagtctgtgctgactcagccaccttcagcatctggtactccaggtcagcgcgtcaccatcagctgccgtggtaacaacatcggtagcaagcgtgtgcattggtatcagcaactcccaggcaccgctcctaagctcctgatttacagctacaaccaccgtcctagcggtgtgcctgatcgcttttctgggtccaagtctggcacctcagcctctctggctatcactggacttcgctccgaggacgaagctgactattactgcaacacttgggacgacagcctggagggtcctgtgttcggcggtgggaccaaactgaccgtccta

SEQ ID NO: 383 - protein, 116 aa, Artificial Sequence
  CB301_H3L1_E6 Heavy Chain Variable Region
EVQLLESGGGLVQPGGSLRLSCAASGFTFSSYAMSWVRQAPGKGLEWVSAISGSGGSTYYADSVKGRFTISRDNSKNTLYLQMNSLRAEDTAVYYCARWHYSFDYWGQGTLVTVSS

SEQ ID NO: 384 - protein, 108 aa, Artificial Sequence
  CB301_H3L1_E6 Light Chain Variable Region
QSVLTQPPSASGTPGQRVTISCRGNNIGSKRVHWYQQLPGTAPKLLIYSYNHRPSGVPDRFSGSKSGTSASLAITGLRSEDEADYYCNTWDDSLEGPVFGGGTKLTVL

SEQ ID NO: 385 - DNA, 352 bp, Artificial Sequence
  CB301_H3L1_F4 Heavy Chain Variable Region
gaggtgcagctgttggagtctggtggaggcttggtacagcctggaggttctcttcgcctctcctgtgcagcctccggattcactttcagcggctacgcaatgagctgggtcagacaggcaccaggtaagggactggagtgggtctctgcaattagcggtagcggtggtagcacttactacgcagacagcgtgaagggtcgcttcaccatctcacgcgacaactccaagaacaccctgtacctgcagatgaacagccttcgcgcagaggacactgccgtgtattactgcgcacgtagtcctagcggtctgttcgactactggggacaaggtactctggtcactgtctcctcag

SEQ ID NO: 386 - DNA, 318 bp, Artificial Sequence
  CB301_H3L1_F4 Light Chain Variable Region
cagtctgtgctgactcagccaccttcagcatctggtactccaggtcagcgcgtcaccatcagctgcggtggtaacaacatcggtagcaagcgtgtgcattggtatcagcaactcccaggcaccgctcctaagctcctgatttacaacactagcaacaagcatagcggtgtgcctgatcgcttttctgggtccaagtctggcacctcagcctctctggctatcagtggacttcgctccgaggacgaggctgactattactgcagcagctacctacagcagcactctctgttcggcggtgggaccaaactaaccgtccta

SEQ ID NO: 387 - protein, 117 aa, Artificial Sequence
  CB301_H3L1_F4 Heavy Chain Variable Region
EVQLLESGGGLVQPGGSLRLSCAASGFTFSGYAMSWVRQAPGKGLEWVSAISGSGGSTYYADSVKGRFTISRDNSKNTLYLQMNSLRAEDTAVYYCARSPSGLFDYWGQGTLVTVSS

SEQ ID NO: 388 - protein, 106 aa, Artificial Sequence
  CB301_H3L1_F4 Light Chain Variable Region
QSVLTQPPSASGTPGQRVTISCGGNNIGSKRVHWYQQLPGTAPKLLIYNTSNKHSGVPDRFSGSKSGTSASLAISGLRSEDEADYYCSSYLQQHSLFGGGTKLTVL

SEQ ID NO: 389 - DNA, 360 bp, Artificial Sequence
  CB301_H3L1_G11 Heavy Chain Variable Region
gaggtgcagctgttggagtctggtggaggcttggtacagcctggaggttcctcttccgcctcctcctgtgcagcctccggattcactttcagcagctacgcaatgagctgggtcagacaggcaccaggtaagggactggagtgggtctctgcaattagcggtagcggtggtagcacttactacgcagacagcgtgaagggtcgcttcaccatctcacgcgacaactccaagaacaccctgtacctgcagatgaacagccttcgcgcagaggacactgccgtgtattactgcacacgtttcgtgggtgcaatcggtgcattcgactactggggacaaggtactctggtcactgtctcctca

SEQ ID NO: 390 - DNA, 324 bp, Artificial Sequence
  CB301_H3L1_G11 Light Chain Variable Region
cagtctgtgctgactcagccaccttcagcatctggtactccaggtcagcgcgtcaccatcagctgcagtggtaacaacatcggtagccgtagcgtgcattggtatcagcaactcccaggcaccgctcctaagctcctgatttaccgcaacaaccagcgccctagtggtgtgcctgatcgcttttctgggtccaagtctggcacctcagcctctctggctatcagtggacttcgctccgaggacgaggctgactattactgcgcagcatgggacgacagcctgagcggtcctgtgttcggcggtgggaccaaactgaccgtccta

SEQ ID NO: 391 - protein, 120 aa, Artificial Sequence
  CB301_H3L1_G11 Heavy Chain Variable Region
EVQLLESGGGLVQPGGSSSASSCAASGFTFSSYAMSWVRQAPGKGLEWVSAISGSGGSTYYADSVKGRFTISRDNSKNTLYLQMNSLRAEDTAVYYCTRFVGAIGAFDYWGQGTLVTVSS

SEQ ID NO: 392 - protein, 108 aa, Artificial Sequence
  CB301_H3L1_G11 Light Chain Variable Region
QSVLTQPPSASGTPGQRVTISCSGNNIGSRSVHWYQQLPGTAPKLLIYRNNQRPSGVPDRFSGSKSGTSASLAISGLRSEDEADYYCAAWDDSLSGPVFGGGTKLTVL

SEQ ID NO: 393 - DNA, 363 bp, Artificial Sequence
  CB301_OPALTL_B5 Heavy Chain Variable Region
gaggtgcagctgttggagtctggtggaggcttggtacagcctggaggttctcttcgcctctcctgtgcagcctccggattcactttcagccattacgcaatgagctgggtcagacaggcaccaggtaagggactggagtgggtctctgcaattagcggtagcggtggtagcacttactacgcagacagcgtgaagggtcgcttcaccatctcacgcgacaactccaagaacaccctgtacctgcagatgaacagccttcgcgcagaggacactgccgtgtattactgcgcacgtggttgggacagccctactctgacatacttcgacagctggggacaaggtactctggtcactgtctcctca

SEQ ID NO: 394 - DNA, 330 bp, Artificial Sequence
  CB301_OPALTL_B5 Light Chain Variable Region
cagtctgtgctgactcagccaccttcagcatctggtactccaggtcagcgcgtcaccatcagctgcagcggtactagcagcaacatcggtaacaacgacgtgagctggtatcagcaactcccaggcaccgctcctaagctcctgatttaccaggacactaagcgtcctagcggtgtgcctgatcgcttttctgggtccaagtctggcacctcagcctctctggctatcagtggacttcgctccgaggacgaggctgactattactgcgcagcatgggacgacagcctgagcggtcctgtgttcggcggtgggaccaaactgaccgtccta

SEQ ID NO: 395 - protein, 121 aa, Artificial Sequence
  CB301_OPALTL_B5 Heavy Chain Variable Region
EVQLLESGGGLVQPGGSLRLSCAASGFTFSHYAMSWVRQAPGKGLEWVSAISGSGGSTYYADSVKGRFTISRDNSKNTLYLQMNSLRAEDTAVYYCARGWDSPTLTYFDSWGQGTLVTVSS

SEQ ID NO: 396 - protein, 110 aa, Artificial Sequence
  CB301_OPALTL_B5 Light Chain Variable Region
QSVLTQPPSASGTPGQRVTISCSGTSSNIGNNDVSWYQQLPGTAPKLLIYQDTKRPSGVPDRFSGSKSGTSASLAISGLRSEDEADYYCAAWDDSLSGPVFGGGTKLTVL

SEQ ID NO: 397 - DNA, 348 bp, Artificial Sequence
  CB301_OPALTL_E6 Heavy Chain Variable Region
gaggtgcagctgttggagtctggtggaggcttggtacagcctggaggttctcttcgcctctcctgtgcagcctccggattcactttcagcagctacggtatgcattgggtcagacaggcaccaggtaagggactggagtgggtctctgcaatcagcggtagcggtggttacacttactacgcagacagcgtgaagggtcgcttcaccatctcacgcgacaactccaagaacaccctgtacctgcagatgaacagccttcgcgcagaggacactgccgtgtattactgcgcacgctggcattacagcttcgactactggggacaaggtactctggtcactgtctcctca

SEQ ID NO: 398 - DNA, 324 bp, Artificial Sequence
  CB301_OPALTL_E6 Light Chain Variable Region
cagtctgtgctgactcagccaccttcagcatctggtactccaggtcagcgcgtcaccatcagctgcagcggtagcagcagcaacatcggtaacaactacgtgagctggtatcagcaactcccaggcaccgctcctaagctcctgatttaccgcaacaaccagcgccctagtggtgtgcctgatcgcttttctgggtccaagtctggcacctcagcctctctggctatcagtggacttcgctccgaggacgaggctgactattactgccagagctacgacaacagcaacgtgctgttcggcggtgggaccaaactgaccgtccta

SEQ ID NO: 399 - protein, 116 aa, Artificial Sequence
  CB301_OPALTL_E6 Heavy Chain Variable Region
EVQLLESGGGLVQPGGSLRLSCAASGFTFSSYGMHWVRQAPGKGLEWVSAISGSGGYTYYADSVKGRFTISRDNSKNTLYLQMNSLRAEDTAVYYCARWHYSFDYWGQGTLVTVSS

SEQ ID NO: 400 - protein, 108 aa, Artificial Sequence
  CB301_OPALTL_E6 Light Chain Variable Region
QSVLTQPPSASGTPGQRVTISCSGSSSNIGNNYVSWYQQLPGTAPKLLIYRNNQRPSGVPDRFSGSKSGTSASLAISGLRSEDEADYYCQSYDNSNVLFGGGTKLTVL

SEQ ID NO: 401 - DNA, 489 bp, Artificial Sequence
  CD300c ECD
ggctattttcctctgagccaccccatgaccgtggcgggccccgtggggggatccctgagtgtgcagtgtcgctatgagaaggaacacaggaccctcaacaaattctggtgcagaccaccacagattctccgatgtgacaagattgtggagaccaaagggtcagcagggaaaaggaatggccgagtgtccatcagggacagtcctgcaaacctcagcttcacagtgaccctggagaatctcacagaggaggacgcaggcacctactggtgtggggtggatacaccgtggctccgagactttcatgatcccattgtcgaggttgaggtgtccgtgttcccggccgggacgaccacagcctccagcccccagagctccatgggcacctcaggtcctcccacgaagctgcccgtgcacacctggcccagcgtgaccagaaaggacagccccgaacccagcccacaccctggctccctgttcagcaatgtccgc

SEQ ID NO: 402 - protein, 163 aa, Artificial Sequence
  CD300c ECD
GYFPLSHPMTVAGPVGGSLSVQCRYEKEHRTLNKFWCRPPQILRCDKIVETKGSAGKRNGRVSIRDSPANLSFTVTLENLTEEDAGTYWCGVDTPWLRDFHDPIVEVEVSVFPAGTTTASSPQSSMGTSGPPTKLPVHTWPSVTRKDSPEPSPHPGSLFSNVR

SEQ ID NO: 403 - protein, 12 aa, Artificial Sequence
  Heavy chain CDR1 of anti-CD300c monoclonal antibody or antigen binding fragment thereof
  MISC_FEATURE (5): Xaa = R, S, or D
  MISC_FEATURE (7): Xaa = A, G, or H
  MISC_FEATURE (9): Xaa = T, H, or S
FTFSXYXMXWVR

SEQ ID NO: 404 - protein, 13 aa, Artificial Sequence
  Heavy chain CDR2 of anti-CD300c monoclonal antibody or antigen binding fragment thereof
  MISC_FEATURE (1): Xaa = S, A, or T
  MISC_FEATURE (2): Xaa = M or I
  MISC_FEATURE (4): Xaa = G or S
  MISC_FEATURE (5): Xaa = T or S
  MISC_FEATURE (8): Xaa = T, S, or Y
  MISC_FEATURE (13): Xaa = D or E
XXSXXGGXTYYAX

SEQ ID NO: 405 - protein, 15 aa, Artificial Sequence
  Heavy chain CDR3 of anti-CD300c monoclonal antibody or antigen binding fragment thereof
  MISC_FEATURE (4): Xaa = R, V, or S
  MISC_FEATURE (5): Xaa = G or S
  MISC_FEATURE (6): Xaa = A, G, S, Y, or I
  MISC_FEATURE (7): Xaa = Y, A, Q, G, or R
  MISC_FEATURE (8): Xaa = G or L
  MISC_FEATURE (9): Xaa = F, R, I, M, or P
  MISC_FEATURE (10): Xaa = D, G, F, or L
  MISC_FEATURE (11): Xaa = H, F, D, or V
  MISC_FEATURE (12): Xaa = F, I, Y, or not present
  MISC_FEATURE (13): Xaa = D or not present
  MISC_FEATURE (14): Xaa = Y or not present
YCAXXXXXXXXXXXW

SEQ ID NO: 406 - protein, 15 aa, Artificial Sequence
  Light chain CDR1 of anti-CD300c monoclonal antibody or antigen binding fragment thereof
  MISC_FEATURE (2): Xaa = R, S, or T
  MISC_FEATURE (3): Xaa = A, G, or R
  MISC_FEATURE (4): Xaa = S or N
  MISC_FEATURE (5): Xaa = Q, S, or N
  MISC_FEATURE (6): Xaa = S, I, or G
  MISC_FEATURE (7): Xaa = I, N, or G
  MISC_FEATURE (8): Xaa = G, I, T, or S
  MISC_FEATURE (9): Xaa = N, G, R, A, or K
  MISC_FEATURE (10): Xaa = Y, S, R, or G
  MISC_FEATURE (11): Xaa = N or not present
  MISC_FEATURE (12): Xaa = Y or not present
  MISC_FEATURE (13): Xaa = L or V
  MISC_FEATURE (14): Xaa = N, Y, H, or Q
CXXXXXXXXXXXXXW

SEQ ID NO: 407 - protein, 10 aa, Artificial Sequence
  Light chain CDR2 of anti-CD300c monoclonal antibody or antigen binding fragment thereof
  MISC_FEATURE (1): Xaa = D, E, S, or R
  MISC_FEATURE (2): Xaa = A, D, K, or N
  MISC_FEATURE (3): Xaa = S or N
  MISC_FEATURE (4): Xaa = N, K, or Q
  MISC_FEATURE (5): Xaa = L or R
  MISC_FEATURE (6): Xaa = E or P
  MISC_FEATURE (7): Xaa = T or S
  MISC_FEATURE (9): Xaa = I or V
  MISC_FEATURE (10): Xaa = P or R
XXXXXXXGXX

SEQ ID NO: 408 - protein, 14 aa, Artificial Sequence
  Light chain CDR3 of anti-CD300c monoclonal antibody or antigen binding fragment thereof
  MISC_FEATURE (3): Xaa = Q, S, or A
  MISC_FEATURE (4): Xaa = Q, S, or A
  MISC_FEATURE (5): Xaa = S, Y, or W
  MISC_FEATURE (6): Xaa = S, T, D, or A
  MISC_FEATURE (7): Xaa = A, S, D, or G
  MISC_FEATURE (8): Xaa = I, S, N, or T
  MISC_FEATURE (9): Xaa = P, S, L, N, or K
  MISC_FEATURE (10): Xaa = Y, T, S, N, or G
  MISC_FEATURE (11): Xaa = V, G, L, or not present
  MISC_FEATURE (12): Xaa  = P or not present
  MISC_FEATURE (13): Xaa = T, I, or V
YCXXXXXXXXXXXF

SEQ ID NO: 409 - DNA, 63 bp, Artificial Sequence
  CD8alpha signal peptide
atggccttaccagtgaccgccttgctcctgccgctggccttgctgctccacgccgccaggccg

SEQ ID NO: 410 - protein, 21 aa, Artificial Sequence
  CD8alpha signal peptide
MALPVTALLLPLALLLHAARP

SEQ ID NO: 411 - DNA, 714 bp, Artificial Sequence
  CK1 scFv
gaagtgcagctgctggaaagtggaggtggactggtgcagcctggcggcagcctgcgcctgagctgtgccgccagcggattcaccttcagccgctatgccatgacctgggttcgccaagcacctggcaaaggcctggaatgggtgagcagcatgagcggcaccggcggcaccacctattatgccgatagcgtgaaaggtcgctttaccatcagccgcgataacagcaaaaacaccctgtatctgcagatgaacagcctgcgcgccgaggacaccgcagtctactactgtgcccgcggcgcctatggctttgatcattggggacaaggtactctggtgaccgtgagcagcagtggaggaggtagcggaggtggtggatctggaggtggaggtagtgaaatcgtgctgacccagagccctggcaccctgagcctgagccctggcgaacgcgcaacactgtcatgccgcgccagccagagcatcggcaactatctgaactggtatcagcagaaaccaggtcaggctccacgtctgctgatctatgatgccagcaacctggaaaccggcatccctgatcgcttctcaggatctggaagcggtaccgattttaccctgaccatcagccgcctggaacctgaggactttgccgtgtattattgtcagcagagtagcgccatcccttataccttcggtcagggcactaaagtggaaatcaaa

SEQ ID NO: 412 - protein, 238 aa, Artificial Sequence
  CK1 scFv
EVQLLESGGGLVQPGGSLRLSCAASGFTFSRYAMTWVRQAPGKGLEWVSSMSGTGGTTYYADSVKGRFTISRDNSKNTLYLQMNSLRAEDTAVYYCARGAYGFDHWGQGTLVTVSSSGGGSGGGGSGGGGSEIVLTQSPGTLSLSPGERATLSCRASQSIGNYLNWYQQKPGQAPRLLIYDASNLETGIPDRFSGSGSGTDFTLTISRLEPEDFAVYYCQQSSAIPYTFGQGTKVEIK

SEQ ID NO: 413 - DNA, 729 bp, Artificial Sequence
  CL6 scFv
gaggtgcagctgttggagtctggtggaggcttggtacagcctggaggttctcttcgcctctcctgtgcagcctccggattcactttcagcagctacggtatgcattgggtcagacaggcaccaggtaagggactggagtgggtctctgcaattagcggtagcggtggtagcacttactacgcagacagcgtgaagggtcgcttcaccatctcacgcgacaactccaagaacaccctgtacctgcagatgaacagccttcgcgcagaggacactgccgtgtattactgcgcagtcagtggtgcaggtcgtggtttcttcgactactggggacaaggtactctggtcactgtctcctcaggtggaggcggttcaggcggaggtggatctggcggtggcggatcccagtctgtgctgactcagccaccttcagcatctggtactccaggtcagcgcgtcaccatcagctgcagcggtagcagcagcaacattggtagcaactacgtgtactggtatcagcaactcccaggcaccgctcctaagctcctgatttacgaggacaacaagcgtcctagtggtgtgcctgatcgcttttctgggtccaagtctggcacctcagcctctctggctatcagtggacttcgctccgaggacgaggctgactattactgcagcagctacactagcagcagcactgtgatcttcggcggtgggaccaaactgaccgtccta

SEQ ID NO: 414 - protein, 243 aa, Artificial Sequence
  CL6 scFv
EVQLLESGGGLVQPGGSLRLSCAASGFTFSSYGMHWVRQAPGKGLEWVSAISGSGGSTYYADSVKGRFTISRDNSKNTLYLQMNSLRAEDTAVYYCAVSGAGRGFFDYWGQGTLVTVSSGGGGSGGGGSGGGGSQSVLTQPPSASGTPGQRVTISCSGSSSNIGSNYVYWYQQLPGTAPKLLIYEDNKRPSGVPDRFSGSKSGTSASLAISGLRSEDEADYYCSSYTSSSTVIFGGGTKLTVL

SEQ ID NO: 415 - DNA, 720 bp, Artificial Sequence
  CL7 scFv
gaggtgcagctgttggagtctggtggaggcttggtacagcctggaggttctcttcgcctctcctgtgcagcctccggattcactttcagccgctacgcaatgagctgggtcagacaggcaccaggtaagggactggagtgggtctctgcaattagcggtagcggtggtagcacttactacgcagacagcgtgaagggtcgcttcaccatctcacgcgacaactccaagaacaccctgtacctgcagatgaacagccttcgcgcagaggacactgccgtgtattactgcgcacgtagcagccagggtatcttcgacatctggggacaaggtactctggtcactgtctcctcaggtggaggcggttcaggcggaggtggatctggcggtggcggatcccagtctgtgctgactcagccaccttcagcatctggtactccaggtcagcgcgtcaccatcagctgcagtggtaacaatatcggtactagacgcgtgcattggtatcagcaactcccagacaccgctcctaagctcctgatttacagtaagaacaaccgtcctagtggtgtgcctgatcgcttttctgggtccaagtctggcacctcagcctctctggctatcagtggacttcgctccgaggacgaggctgactattactgcgcagcatgggacgacagcctgagcggtcctgtgttcggcggtgggaccaaactgaccgtccta

SEQ ID NO: 416 - protein, 240 aa, Artificial Sequence
  CL7 scFv
EVQLLESGGGLVQPGGSLRLSCAASGFTFSRYAMSWVRQAPGKGLEWVSAISGSGGSTYYADSVKGRFTISRDNSKNTLYLQMNSLRAEDTAVYYCARSSQGIFDIWGQGTLVTVSSGGGGSGGGGSGGGGSQSVLTQPPSASGTPGQRVTISCSGNNIGTRRVHWYQQLPDTAPKLLIYSKNNRPSGVPDRFSGSKSGTSASLAISGLRSEDEADYYCAAWDDSLSGPVFGGGTKLTVL

SEQ ID NO: 417 - DNA, 720 bp, Artificial Sequence
  CL10 scFv
gaggtgcagctgttggagtctggtggaggcttggtacagcctggaggttctcttcgcctctcctgtgcagcctccggattcactttcagcagctacggtatgcattgggtcagacaggcaccaggtaagggactggagtgggtctctgcaattagcggtagcggtggtagcacttactacgcagacagcgtgaagggtcgcttcaccatctcacgcgacaactccaagaacaccctgtacctgcagatgaacagccttcgcgcagaggacactgccgtgtattactgcgcaagcggttacggtctgatggacgtgtggggacaaggtactctggtcactgtctcctcaggtggaggcggttcaggcggaggtggatctggcggtggcggatcccagtctgtgctgactcagccaccttcagcatctggtactccaggtcagcgcgtcaccatcagctgcactcgtagcagcggtatcatcgcaagcaactacgtgcagtggtatcagcaactcccaggcaccgctcctaagctcctgatttaccgcaacaaccagcgccctagtggtgtgcctgatcgcttttctgggtccaagtctggcacctcagcctctctggctatcagtggacttcgctccgaggacgaggctgactattactgcagcagctacgcaggtaacaacaacctggtgttcggcggtgggaccaaactgaccgtccta

SEQ ID NO: 418 - protein, 240 aa, Artificial Sequence
  CL10 scFv
EVQLLESGGGLVQPGGSLRLSCAASGFTFSSYGMHWVRQAPGKGLEWVSAISGSGGSTYYADSVKGRFTISRDNSKNTLYLQMNSLRAEDTAVYYCASGYGLMDVWGQGTLVTVSSGGGGSGGGGSGGGGSQSVLTQPPSASGTPGQRVTISCTRSSGIIASNYVQWYQQLPGTAPKLLIYRNNQRPSGVPDRFSGSKSGTSASLAISGLRSEDEADYYCSSYAGNNNLVFGGGTKLTVL

SEQ ID NO: 419 - DNA, 717 bp, Artificial Sequence
  SL18 scFv
cgagtgcagctgctggaaagtggaggtggactggtgcagcctggcggcagcctgcgcctgagctgtgccgccagcggattcaccttcagcgattatcatatgcattgggttcgccaagcacctggcaaaggcctggaatgggtgagcaccatcagcagcagcggcggctatacctattatgccgaaagcgtgaaaagccgctttaccatcagccgcgataacagcaaaaacaccctgtatctgcagatgaacagcctgcgcgccgaggacaccgcagtctactactgtgcccgatcgatacgcctgcctctggattattggggacaaggtactctggtgaccgtgagcagcagtggaggaggtagcggaggtggtggatctggaggtggaggtagtcagagcgtgctgacccagcctcctagcgcctccggtacaccaggacagcgcgtgactattagctgtagcggcaacaacatcggcagcaaaggcgtgcattggtatcagcaactgcctggaactgcacctaagctgctgatctatgaagatagcaaacgccctagcggcgtgcgtgatcgctttagcggtagcaaatcaggcaccagcgccagcctggccatcagcggccttcgctccgaagatgaagccgattattattgtcagagctatgatagcaccaaaggcgtggtgtttggtggcggtaccaagctgaccgtgctg

SEQ ID NO: 420 - protein, 239 aa, Artificial Sequence
  SL18 scFv
RVQLLESGGGLVQPGGSLRLSCAASGFTFSDYHMHWVRQAPGKGLEWVSTISSSGGYTYYAESVKSRFTISRDNSKNTLYLQMNSLRAEDTAVYYCARSIRLPLDYWGQGTLVTVSSSGGGSGGGGSGGGGSQSVLTQPPSASGTPGQRVTISCSGNNIGSKGVHWYQQLPGTAPKLLIYEDSKRPSGVRDRFSGSKSGTSASLAISGLRSEDEADYYCQSYDSTKGVVFGGGTKLTVL

SEQ ID NO: 421 - DNA, 30 bp, Artificial Sequence
  GS linker
ggtggcggaggttctggaggtggaggttcc

SEQ ID NO: 422 - protein, 10 aa, Artificial Sequence
  GS linker
GGGGSGGGGS

SEQ ID NO: 423 - DNA, 135 bp, Artificial Sequence
  CD8 hinge
accacgacgccagcgccgcgaccaccaacaccggcgcccaccatcgcgtcgcagcccctgtccctgcgcccagaggcgtgccggccagcggcggggggcgcagtgcacacgagggggctggacttcgcctgtgat

SEQ ID NO: 424 - protein, 45 aa, Artificial Sequence
  CD8 hinge
TTTPAPRPPTPAPTIASQPLSLRPEACRPAAGGAVHTRGLDFACD

SEQ ID NO: 425 - DNA, 81 bp, Artificial Sequence
  CD28 transmembrane domain
ttttgggtgctggtggtggttggtggagtcctggcttgctatagcttgctagtaacagtggcctttattattttctgggtg

SEQ ID NO: 426 - protein, 27 aa, Artificial Sequence
  CD28 transmembrane domain
FWVLVVVGGVLACYSLLVTVAFIIFWV

SEQ ID NO: 427 - DNA, 123 bp, Artificial Sequence
  CD28 intracellular domain
aggagtaagaggagcaggctcctgcacagtgactacatgaacatgactccccgccgccccgggcccacccgcaagcattaccagccctatgccccaccacgcgacttcgcagcctatcgctcc

SEQ ID NO: 428 - protein, 41 aa, Artificial Sequence
  CD28 intracellular domain
RSKRSRLLHSDYMNMTPRRPGPTRKHYQPYAPPRDFAAYRS

SEQ ID NO: 429 - DNA, 339 bp, Artificial Sequence
  CD3zeta intracellular domain
agagtgaagttcagcaggagcgcagacgcccccgcgtaccagcagggccagaaccagctctataacgagctcaatctaggacgaagagaggagtacgatgttttggacaagagacgtggccgggaccctgagatggggggaaagccgagaaggaagaaccctcaggaaggcctgtacaatgaactgcagaaagataagatggcggaggcctacagtgagattgggatgaaaggcgagcgccggaggggcaaggggcacgatggcctttaccagggtctcagtacagccaccaaggacacctacgacgcccttcacatgcaggccctgccccctcgctaa

SEQ ID NO: 430 - protein, 112 aa, Artificial Sequence
  CD3zeta intracellular domain
RVKFSRSADAPAYQQGQNQLYNELNLGRREEYDVLDKRRGRDPEMGGKPRRKNPQEGLYNELQKDKMAEAYSEIGMKGERRRGKGHDGLYQGLSTATKDTYDALHMQALPPR

SEQ ID NO: 431 - DNA, 1485 bp, Artificial Sequence
  CK1 CAR
atggccttaccagtgaccgccttgctcctgccgctggccttgctgctccacgccgccaggccggaagtgcagctgctggaaagtggaggtggactggtgcagcctggcggcagcctgcgcctgagctgtgccgccagcggattcaccttcagccgctatgccatgacctgggttcgccaagcacctggcaaaggcctggaatgggtgagcagcatgagcggcaccggcggcaccacctattatgccgatagcgtgaaaggtcgctttaccatcagccgcgataacagcaaaaacaccctgtatctgcagatgaacagcctgcgcgccgaggacaccgcagtctactactgtgcccgcggcgcctatggctttgatcattggggacaaggtactctggtgaccgtgagcagcagtggaggaggtagcggaggtggtggatctggaggtggaggtagtgaaatcgtgctgacccagagccctggcaccctgagcctgagccctggcgaacgcgcaacactgtcatgccgcgccagccagagcatcggcaactatctgaactggtatcagcagaaaccaggtcaggctccacgtctgctgatctatgatgccagcaacctggaaaccggcatccctgatcgcttctcaggatctggaagcggtaccgattttaccctgaccatcagccgcctggaacctgaggactttgccgtgtattattgtcagcagagtagcgccatcccttataccttcggtcagggcactaaagtggaaatcaaaggtggcggaggttctggaggtggaggttccaccacgacgccagcgccgcgaccaccaacaccggcgcccaccatcgcgtcgcagcccctgtccctgcgcccagaggcgtgccggccagcggcggggggcgcagtgcacacgagggggctggacttcgcctgtgatttttgggtgctggtggtggttggtggagtcctggcttgctatagcttgctagtaacagtggcctttattattttctgggtgaggagtaagaggagcaggctcctgcacagtgactacatgaacatgactccccgccgccccgggcccacccgcaagcattaccagccctatgccccaccacgcgacttcgcagcctatcgctccagagtgaagttcagcaggagcgcagacgcccccgcgtaccagcagggccagaaccagctctataacgagctcaatctaggacgaagagaggagtacgatgttttggacaagagacgtggccgggaccctgagatggggggaaagccgagaaggaagaaccctcaggaaggcctgtacaatgaactgcagaaagataagatggcggaggcctacagtgagattgggatgaaaggcgagcgccggaggggcaaggggcacgatggcctttaccagggtctcagtacagccaccaaggacacctacgacgcccttcacatgcaggccctgccccctcgctaa

SEQ ID NO: 432 - protein, 494 aa, Artificial Sequence
  CK1 CAR
MALPVTALLLPLALLLHAARPEVQLLESGGGLVQPGGSLRLSCAASGFTFSRYAMTWVRQAPGKGLEWVSSMSGTGGTTYYADSVKGRFTISRDNSKNTLYLQMNSLRAEDTAVYYCARGAYGFDHWGQGTLVTVSSSGGGSGGGGSGGGGSEIVLTQSPGTLSLSPGERATLSCRASQSIGNYLNWYQQKPGQAPRLLIYDASNLETGIPDRFSGSGSGTDFTLTISRLEPEDFAVYYCQQSSAIPYTFGQGTKVEIKGGGGSGGGGSTTTPAPRPPTPAPTIASQPLSLRPEACRPAAGGAVHTRGLDFACDFWVLVVVGGVLACYSLLVTVAFIIFWVRSKRSRLLHSDYMNMTPRRPGPTRKHYQPYAPPRDFAAYRSRVKFSRSADAPAYQQGQNQLYNELNLGRREEYDVLDKRRGRDPEMGGKPRRKNPQEGLYNELQKDKMAEAYSEIGMKGERRRGKGHDGLYQGLSTATKDTYDALHMQALPPR

SEQ ID NO: 433 - DNA, 1500 bp, Artificial Sequence
  CL6 CAR
atggccttaccagtgaccgccttgctcctgccgctggccttgctgctccacgccgccaggccggaggtgcagctgttggagtctggtggaggcttggtacagcctggaggttctcttcgcctctcctgtgcagcctccggattcactttcagcagctacggtatgcattgggtcagacaggcaccaggtaagggactggagtgggtctctgcaattagcggtagcggtggtagcacttactacgcagacagcgtgaagggtcgcttcaccatctcacgcgacaactccaagaacaccctgtacctgcagatgaacagccttcgcgcagaggacactgccgtgtattactgcgcagtcagtggtgcaggtcgtggtttcttcgactactggggacaaggtactctggtcactgtctcctcaggtggaggcggttcaggcggaggtggatctggcggtggcggatcccagtctgtgctgactcagccaccttcagcatctggtactccaggtcagcgcgtcaccatcagctgcagcggtagcagcagcaacattggtagcaactacgtgtactggtatcagcaactcccaggcaccgctcctaagctcctgatttacgaggacaacaagcgtcctagtggtgtgcctgatcgcttttctgggtccaagtctggcacctcagcctctctggctatcagtggacttcgctccgaggacgaggctgactattactgcagcagctacactagcagcagcactgtgatcttcggcggtgggaccaaactgaccgtcctaggtggcggaggttctggaggtggaggttccaccacgacgccagcgccgcgaccaccaacaccggcgcccaccatcgcgtcgcagcccctgtccctgcgcccagaggcgtgccggccagcggcggggggcgcagtgcacacgagggggctggacttcgcctgtgatttttgggtgctggtggtggttggtggagtcctggcttgctatagcttgctagtaacagtggcctttattattttctgggtgaggagtaagaggagcaggctcctgcacagtgactacatgaacatgactccccgccgccccgggcccacccgcaagcattaccagccctatgccccaccacgcgacttcgcagcctatcgctccagagtgaagttcagcaggagcgcagacgcccccgcgtaccagcagggccagaaccagctctataacgagctcaatctaggacgaagagaggagtacgatgttttggacaagagacgtggccgggaccctgagatggggggaaagccgagaaggaagaaccctcaggaaggcctgtacaatgaactgcagaaagataagatggcggaggcctacagtgagattgggatgaaaggcgagcgccggaggggcaaggggcacgatggcctttaccagggtctcagtacagccaccaaggacacctacgacgcccttcacatgcaggccctgccccctcgctaa

SEQ ID NO: 434 - protein, 499 aa, Artificial Sequence
  CL6 CAR
MALPVTALLLPLALLLHAARPEVQLLESGGGLVQPGGSLRLSCAASGFTFSSYGMHWVRQAPGKGLEWVSAISGSGGSTYYADSVKGRFTISRDNSKNTLYLQMNSLRAEDTAVYYCAVSGAGRGFFDYWGQGTLVTVSSGGGGSGGGGSGGGGSQSVLTQPPSASGTPGQRVTISCSGSSSNIGSNYVYWYQQLPGTAPKLLIYEDNKRPSGVPDRFSGSKSGTSASLAISGLRSEDEADYYCSSYTSSSTVIFGGGTKLTVLGGGGSGGGGSTTTPAPRPPTPAPTIASQPLSLRPEACRPAAGGAVHTRGLDFACDFWVLVVVGGVLACYSLLVTVAFIIFWVRSKRSRLLHSDYMNMTPRRPGPTRKHYQPYAPPRDFAAYRSRVKFSRSADAPAYQQGQNQLYNELNLGRREEYDVLDKRRGRDPEMGGKPRRKNPQEGLYNELQKDKMAEAYSEIGMKGERRRGKGHDGLYQGLSTATKDTYDALHMQALPPR

SEQ ID NO: 435 - DNA, 1491 bp, Artificial Sequence
  CL7 CAR
atggccttaccagtgaccgccttgctcctgccgctggccttgctgctccacgccgccaggccggaggtgcagctgttggagtctggtggaggcttggtacagcctggaggttctcttcgcctctcctgtgcagcctccggattcactttcagccgctacgcaatgagctgggtcagacaggcaccaggtaagggactggagtgggtctctgcaattagcggtagcggtggtagcacttactacgcagacagcgtgaagggtcgcttcaccatctcacgcgacaactccaagaacaccctgtacctgcagatgaacagccttcgcgcagaggacactgccgtgtattactgcgcacgtagcagccagggtatcttcgacatctggggacaaggtactctggtcactgtctcctcaggtggaggcggttcaggcggaggtggatctggcggtggcggatcccagtctgtgctgactcagccaccttcagcatctggtactccaggtcagcgcgtcaccatcagctgcagtggtaacaatatcggtactagacgcgtgcattggtatcagcaactcccagacaccgctcctaagctcctgatttacagtaagaacaaccgtcctagtggtgtgcctgatcgcttttctgggtccaagtctggcacctcagcctctctggctatcagtggacttcgctccgaggacgaggctgactattactgcgcagcatgggacgacagcctgagcggtcctgtgttcggcggtgggaccaaactgaccgtcctaggtggcggaggttctggaggtggaggttccaccacgacgccagcgccgcgaccaccaacaccggcgcccaccatcgcgtcgcagcccctgtccctgcgcccagaggcgtgccggccagcggcggggggcgcagtgcacacgagggggctggacttcgcctgtgatttttgggtgctggtggtggttggtggagtcctggcttgctatagcttgctagtaacagtggcctttattattttctgggtgaggagtaagaggagcaggctcctgcacagtgactacatgaacatgactccccgccgccccgggcccacccgcaagcattaccagccctatgccccaccacgcgacttcgcagcctatcgctccagagtgaagttcagcaggagcgcagacgcccccgcgtaccagcagggccagaaccagctctataacgagctcaatctaggacgaagagaggagtacgatgttttggacaagagacgtggccgggaccctgagatggggggaaagccgagaaggaagaaccctcaggaaggcctgtacaatgaactgcagaaagataagatggcggaggcctacagtgagattgggatgaaaggcgagcgccggaggggcaaggggcacgatggcctttaccagggtctcagtacagccaccaaggacacctacgacgcccttcacatgcaggccctgccccctcgctaa

SEQ ID NO: 436 - protein, 496 aa, Artificial Sequence
  CL7 CAR
MALPVTALLLPLALLLHAARPEVQLLESGGGLVQPGGSLRLSCAASGFTFSRYAMSWVRQAPGKGLEWVSAISGSGGSTYYADSVKGRFTISRDNSKNTLYLQMNSLRAEDTAVYYCARSSQGIFDIWGQGTLVTVSSGGGGSGGGGSGGGGSQSVLTQPPSASGTPGQRVTISCSGNNIGTRRVHWYQQLPDTAPKLLIYSKNNRPSGVPDRFSGSKSGTSASLAISGLRSEDEADYYCAAWDDSLSGPVFGGGTKLTVLGGGGSGGGGSTTTPAPRPPTPAPTIASQPLSLRPEACRPAAGGAVHTRGLDFACDFWVLVVVGGVLACYSLLVTVAFIIFWVRSKRSRLLHSDYMNMTPRRPGPTRKHYQPYAPPRDFAAYRSRVKFSRSADAPAYQQGQNQLYNELNLGRREEYDVLDKRRGRDPEMGGKPRRKNPQEGLYNELQKDKMAEAYSEIGMKGERRRGKGHDGLYQGLSTATKDTYDALHMQALPPR

SEQ ID NO: 437 - DNA, 1491 bp, Artificial Sequence
  CL10 CAR
atggccttaccagtgaccgccttgctcctgccgctggccttgctgctccacgccgccaggccggaggtgcagctgttggagtctggtggaggcttggtacagcctggaggttctcttcgcctctcctgtgcagcctccggattcactttcagcagctacggtatgcattgggtcagacaggcaccaggtaagggactggagtgggtctctgcaattagcggtagcggtggtagcacttactacgcagacagcgtgaagggtcgcttcaccatctcacgcgacaactccaagaacaccctgtacctgcagatgaacagccttcgcgcagaggacactgccgtgtattactgcgcaagcggttacggtctgatggacgtgtggggacaaggtactctggtcactgtctcctcaggtggaggcggttcaggcggaggtggatctggcggtggcggatcccagtctgtgctgactcagccaccttcagcatctggtactccaggtcagcgcgtcaccatcagctgcactcgtagcagcggtatcatcgcaagcaactacgtgcagtggtatcagcaactcccaggcaccgctcctaagctcctgatttaccgcaacaaccagcgccctagtggtgtgcctgatcgcttttctgggtccaagtctggcacctcagcctctctggctatcagtggacttcgctccgaggacgaggctgactattactgcagcagctacgcaggtaacaacaacctggtgttcggcggtgggaccaaactgaccgtcctaggtggcggaggttctggaggtggaggttccaccacgacgccagcgccgcgaccaccaacaccggcgcccaccatcgcgtcgcagcccctgtccctgcgcccagaggcgtgccggccagcggcggggggcgcagtgcacacgagggggctggacttcgcctgtgatttttgggtgctggtggtggttggtggagtcctggcttgctatagcttgctagtaacagtggcctttattattttctgggtgaggagtaagaggagcaggctcctgcacagtgactacatgaacatgactccccgccgccccgggcccacccgcaagcattaccagccctatgccccaccacgcgacttcgcagcctatcgctccagagtgaagttcagcaggagcgcagacgcccccgcgtaccagcagggccagaaccagctctataacgagctcaatctaggacgaagagaggagtacgatgttttggacaagagacgtggccgggaccctgagatggggggaaagccgagaaggaagaaccctcaggaaggcctgtacaatgaactgcagaaagataagatggcggaggcctacagtgagattgggatgaaaggcgagcgccggaggggcaaggggcacgatggcctttaccagggtctcagtacagccaccaaggacacctacgacgcccttcacatgcaggccctgccccctcgctaa

SEQ ID NO: 438 - protein, 496 aa, Artificial Sequence
  CL10 CAR
MALPVTALLLPLALLLHAARPEVQLLESGGGLVQPGGSLRLSCAASGFTFSSYGMHWVRQAPGKGLEWVSAISGSGGSTYYADSVKGRFTISRDNSKNTLYLQMNSLRAEDTAVYYCASGYGLMDVWGQGTLVTVSSGGGGSGGGGSGGGGSQSVLTQPPSASGTPGQRVTISCTRSSGIIASNYVQWYQQLPGTAPKLLIYRNNQRPSGVPDRFSGSKSGTSASLAISGLRSEDEADYYCSSYAGNNNLVFGGGTKLTVLGGGGSGGGGSTTTPAPRPPTPAPTIASQPLSLRPEACRPAAGGAVHTRGLDFACDFWVLVVVGGVLACYSLLVTVAFIIFWVRSKRSRLLHSDYMNMTPRRPGPTRKHYQPYAPPRDFAAYRSRVKFSRSADAPAYQQGQNQLYNELNLGRREEYDVLDKRRGRDPEMGGKPRRKNPQEGLYNELQKDKMAEAYSEIGMKGERRRGKGHDGLYQGLSTATKDTYDALHMQALPPR

SEQ ID NO: 439 - DNA, 1488 bp, Artificial Sequence
  SL18 CAR
atggccttaccagtgaccgccttgctcctgccgctggccttgctgctccacgccgccaggccgcgagtgcagctgctggaaagtggaggtggactggtgcagcctggcggcagcctgcgcctgagctgtgccgccagcggattcaccttcagcgattatcatatgcattgggttcgccaagcacctggcaaaggcctggaatgggtgagcaccatcagcagcagcggcggctatacctattatgccgaaagcgtgaaaagccgctttaccatcagccgcgataacagcaaaaacaccctgtatctgcagatgaacagcctgcgcgccgaggacaccgcagtctactactgtgcccgatcgatacgcctgcctctggattattggggacaaggtactctggtgaccgtgagcagcagtggaggaggtagcggaggtggtggatctggaggtggaggtagtcagagcgtgctgacccagcctcctagcgcctccggtacaccaggacagcgcgtgactattagctgtagcggcaacaacatcggcagcaaaggcgtgcattggtatcagcaactgcctggaactgcacctaagctgctgatctatgaagatagcaaacgccctagcggcgtgcgtgatcgctttagcggtagcaaatcaggcaccagcgccagcctggccatcagcggccttcgctccgaagatgaagccgattattattgtcagagctatgatagcaccaaaggcgtggtgtttggtggcggtaccaagctgaccgtgctgggtggcggaggttctggaggtggaggttccaccacgacgccagcgccgcgaccaccaacaccggcgcccaccatcgcgtcgcagcccctgtccctgcgcccagaggcgtgccggccagcggcggggggcgcagtgcacacgagggggctggacttcgcctgtgatttttgggtgctggtggtggttggtggagtcctggcttgctatagcttgctagtaacagtggcctttattattttctgggtgaggagtaagaggagcaggctcctgcacagtgactacatgaacatgactccccgccgccccgggcccacccgcaagcattaccagccctatgccccaccacgcgacttcgcagcctatcgctccagagtgaagttcagcaggagcgcagacgcccccgcgtaccagcagggccagaaccagctctataacgagctcaatctaggacgaagagaggagtacgatgttttggacaagagacgtggccgggaccctgagatggggggaaagccgagaaggaagaaccctcaggaaggcctgtacaatgaactgcagaaagataagatggcggaggcctacagtgagattgggatgaaaggcgagcgccggaggggcaaggggcacgatggcctttaccagggtctcagtacagccaccaaggacacctacgacgcccttcacatgcaggccctgccccctcgctaa

SEQ ID NO: 440 - protein, 495 aa, Artificial Sequence
  SL18 CAR
MALPVTALLLPLALLLHAARPRVQLLESGGGLVQPGGSLRLSCAASGFTFSDYHMHWVRQAPGKGLEWVSTISSSGGYTYYAESVKSRFTISRDNSKNTLYLQMNSLRAEDTAVYYCARSIRLPLDYWGQGTLVTVSSSGGGSGGGGSGGGGSQSVLTQPPSASGTPGQRVTISCSGNNIGSKGVHWYQQLPGTAPKLLIYEDSKRPSGVRDRFSGSKSGTSASLAISGLRSEDEADYYCQSYDSTKGVVFGGGTKLTVLGGGGSGGGGSTTTPAPRPPTPAPTIASQPLSLRPEACRPAAGGAVHTRGLDFACDFWVLVVVGGVLACYSLLVTVAFIIFWVRSKRSRLLHSDYMNMTPRRPGPTRKHYQPYAPPRDFAAYRSRVKFSRSADAPAYQQGQNQLYNELNLGRREEYDVLDKRRGRDPEMGGKPRRKNPQEGLYNELQKDKMAEAYSEIGMKGERRRGKGHDGLYQGLSTATKDTYDALHMQALPPR

SEQ ID NO: 441 - DNA, 1260 bp, Artificial Sequence
  CD300c ECD CAR
atggccttaccagtgaccgccttgctcctgccgctggccttgctgctccacgccgccaggccgggctattttcctctgagccaccccatgaccgtggcgggccccgtggggggatccctgagtgtgcagtgtcgctatgagaaggaacacaggaccctcaacaaattctggtgcagaccaccacagattctccgatgtgacaagattgtggagaccaaagggtcagcagggaaaaggaatggccgagtgtccatcagggacagtcctgcaaacctcagcttcacagtgaccctggagaatctcacagaggaggacgcaggcacctactggtgtggggtggatacaccgtggctccgagactttcatgatcccattgtcgaggttgaggtgtccgtgttcccggccgggacgaccacagcctccagcccccagagctccatgggcacctcaggtcctcccacgaagctgcccgtgcacacctggcccagcgtgaccagaaaggacagccccgaacccagcccacaccctggctccctgttcagcaatgtccgcggtggcggaggttctggaggtggaggttccaccacgacgccagcgccgcgaccaccaacaccggcgcccaccatcgcgtcgcagcccctgtccctgcgcccagaggcgtgccggccagcggcggggggcgcagtgcacacgagggggctggacttcgcctgtgatttttgggtgctggtggtggttggtggagtcctggcttgctatagcttgctagtaacagtggcctttattattttctgggtgaggagtaagaggagcaggctcctgcacagtgactacatgaacatgactccccgccgccccgggcccacccgcaagcattaccagccctatgccccaccacgcgacttcgcagcctatcgctccagagtgaagttcagcaggagcgcagacgcccccgcgtaccagcagggccagaaccagctctataacgagctcaatctaggacgaagagaggagtacgatgttttggacaagagacgtggccgggaccctgagatggggggaaagccgagaaggaagaaccctcaggaaggcctgtacaatgaactgcagaaagataagatggcggaggcctacagtgagattgggatgaaaggcgagcgccggaggggcaaggggcacgatggcctttaccagggtctcagtacagccaccaaggacacctacgacgcccttcacatgcaggccctgccccctcgctaa

SEQ ID NO: 442 - protein, 419 aa, Artificial Sequence
  CD300c ECD CAR
MALPVTALLLPLALLLHAARPGYFPLSHPMTVAGPVGGSLSVQCRYEKEHRTLNKFWCRPPQILRCDKIVETKGSAGKRNGRVSIRDSPANLSFTVTLENLTEEDAGTYWCGVDTPWLRDFHDPIVEVEVSVFPAGTTTASSPQSSMGTSGPPTKLPVHTWPSVTRKDSPEPSPHPGSLFSNVRGGGGSGGGGSTTTPAPRPPTPAPTIASQPLSLRPEACRPAAGGAVHTRGLDFACDFWVLVVVGGVLACYSLLVTVAFIIFWVRSKRSRLLHSDYMNMTPRRPGPTRKHYQPYAPPRDFAAYRSRVKFSRSADAPAYQQGQNQLYNELNLGRREEYDVLDKRRGRDPEMGGKPRRKNPQEGLYNELQKDKMAEAYSEIGMKGERRRGKGHDGLYQGLSTATKDTYDALHMQALPPR